European Patent Application EP 4 417 261 A2, published August 21, 2024. Title: Bacteriotherapy. Applicant: Genome Research Limited. Application GB. The sequence listing filed with the application follows.

SEQUENCE LISTING (51 sequences)

SEQ ID NO: 1 - DNA, 1467 bp, HMI 1 Clostridium thermocellum 16S rDNA
  source 1..1467: mol_type = genomic DNA
caggacgaacgctggcggcgtgcctaacacatgcaagtcgaacgagaatctttgaacagatcttttcggagtgacgttcaaagaggaaagtggcggacgggcgagtaacgcgtgagtaacctgcccataagagggggataatccatggaaacgtggactaataccgcatattgtagtcaagtcgcatgactagattatgaaagatttatcgcttatggatggactcgcgtcagattagatagttggtgaggtaacggctcaccaagtcaacgatctgtagccgaactgagaggttgatcggccgcattgggactgagacacggcccagactcctacgggaggcagcagtggggaatattgcgcaatgggggcaaccctgacgcagcaacgccgcgtgcaggaagaaggtcttcggattgtaaactgttgtcgcaagggaagaagacagtgacggtaccttgtgagaaagtcacggctaactacgtgccagcagccgcggtaatacgtaggtgacaagcgttgtccggatttactgggtgtaaagggcgcgtaggcggactgtcaagtcagtcgtgaaataccggggcttaaccccggggctgcgattgaaactgacagccttgagtatcggagaggaaagcggaattcctagtgtagcggtgaaatgcgtagatattaggaggaacaccagtggcgaaggcggctttctggacgacaactgacgctgaggcgcgaaagtgtggggagcaaacaggattagataccctggtagtccacaccgtaaacgatggatactaggtgtaggaggtatcgaccccttctgtgccgcagttaacacaataagtatcccacctggggagtacgaccgcaaggttgaaactcaaaggaattgacgggggcccgcacaagcagtggagtatgtggtttaattcgaagcaacgcgaagaaccttacctgggcttgacatccctggaatcgagtagagatacttgagtgccttcgggaatcaggtgacaggtggtgcatggttgtcgtcagctcgtgtcgtgagatgttgggttaagtcccgcaacgagcgcaacccctattgtcagttgccatcattaagttgggcactctggcgagactgccggtgacaaatcggaggaaggtggggacgacgtcaaatcatcatgccccttatgcccagggctacacacgtactacaatggccgataacaaagtgcagcgaaaccgtgaggtggagcgaatcacaaaactcggtctcagttcagattgcaggctgcaactcgcctgcatgaagttggaattgctagtaatcgcggatcagaatgccgcggtgaatacgttcccgggccttgtacacaccgcccgtcacaccatgagagtcgataacacccgaagcctgtgagctaacctattaggaggcagcagtcgaaggtggggttgatgattggggtgaagtcg

SEQ ID NO: 2 - DNA, 1419 bp, HMI 2 Flavonifractor pautii 16S rDNA
  source 1..1419: mol_type = genomic DNA
gagtgctcatgacagaggattcgtccaatggagtgagttacttagtggcggacgggtgagtaacgcgtgagtaacctgccttggagtggggaataacaggtggaaacatctgctaataccgcatgatgcagttgggtcgcatggctctgactgccaaagatttatcgctctgagatggactcgcgtctgattagctggttggcggggtaacggcccaccaaggcgacgatcagtagccggactgagaggttggccggccacattgggactgagacacggcccagactcctacgggaggcagcagtggggaatattgggcaatgggcgcaagcctgacccagcaacgccgcgtgaaggaagaaggctttcgggttgtaaacttcttttctcagggacgaagcaagtgacggtacctgaggaataagccacggctaactacgtgccagcagccgcggtaatacgtaggtggcgagcgttatccggatttactgggtgtaaagggcgtgtaggcgggactgcaagtcagatgtgaaaaccatgggctcaacctgtggcctgcatttgaaactgtagttcttgagtactggagaggcagacggaattcctagtgtagcggtgaaatgcgtagatattaggaggaacaccagtggcgaaggcggtctgctggacagcaactgacgctgaggcgcgaaagcgtggggagcaaacaggattagataccctggtagtccacgctgtaaacgatggatactaggtgtggggggtctgaccccctccgtgccgcagttaacacaataagtatcccacctggggagtacgatcgcaaggttgaaactcaaaggaattgacgggggcccgcacaagcggtggagtatgtggtttaattcgaagcaacgcgaagaaccttaccagggcttgacatcccggtgaccggtgtagagatacaccttcttcttcggaagcgccggtgacaggtggtgcatggttgtcgtcagctcgtgtcgtgagatgttgggttaagtcccgcaacgagcgcaacccttattgttagttgctacgcaagagcactctagcgagactgccgttgacaaaacggaggaaggtggggacgacgtcaaatcatcatgccccttatgtcctgggccacacacgtactacaatggtggtcaacagagggaagcaagaccgcgaggtggagcaaacccctaaaagccatcccagttcggattgcaggctgcaactcgcctgtatgaagttggaatcgctagtaatcgcggatcagcatgccgcggtgaatacgttcccgggccttgtacacaccgcccgtcacaccatgagagtcgggaacacccgaagtccgtagcctaaccgcaaggggggcgcggccgaaggtgggttcgataattggggtgaagtcgt

SEQ ID NO: 3 - DNA, 1398 bp, HMI 3 Flavonifractor plautii 16S rDNA
  source 1..1398: mol_type = genomic DNA
tggctgtttagtggcggacgggtgagtaacgcgtgagtaacctgccttggagtggggaataacacagtgaaaactgtgctaataccgcatgacatattggtgtcgcatggcactgatatcaaagatttatcgctctgagatggactcgcgtctgattagatagttggcggggtaacggcccaccaagtcgacgatcagtagccggactgagaggttggccggccacattgggactgagacacggcccagactcctacgggaggcagcagtggggaatattgggcaatgggcgcaagcctgacccagcaacgccgcgtgaaggaagaaggctttcgggttgtaaacttcttttaacagggacgaagtaagtgacggtacctgttgaataagccacggctaactacgtgccagcagccgcggtaatacgtaggtggcaagcgttatccggatttactgggtgtaaagggcgtgtaggcgggactgcaagtcagatgtgaaaactatgggctcaacccatagcctgcatttgaaactgtagttcttgagtgtcggagaggcaatcggaattccgtgtgtagcggtgaaatgcgtagatatacggaggaacaccagtggcgaaggcggattgctggacgataactgacgctgaggcgcgaaagcgtggggagcaaacaggattagataccctggtagtccacgccgtaaacgatggatactaggtgtggggggtctgaccccctccgtgccgcagctaacgcaataagtatcccacctggggagtacgatcgcaaggttgaaactcaaaggaattgacgggggcccgcacaagcggtggagtatgtggtttaattcgaagcaacgcgaagaaccttaccagggcttgacatcctactaacgaaccagagatggattaggtgcccttcggggaaagtagagacaggtggtgcatggttgtcgtcagctcgtgtcgtgagatgttgggttaagtcccgcaacgagcgcaacccttattgttagttgctacgcaagagcactctagcgagactgccgttgacaaaacggaggaaggtggggacgacgtcaaatcatcatgccccttatgtcctgggccacacacgtactacaatggcggttaacagagggaggcaaagccgcgaggcagagcaaacccctaaaagccgtcccagttcggattgcaggctgaaacccgcctgtatgaagtcggaatcgctagtaatcgcggatcagcatgccgcggtgaatacgttcccgggccttgtacacaccgcccgtcacaccatgagagtcgggaacacccgaagtccgtagcctaactgcaaagggggcgcggccgaaggtgggttcgataattggggtgaagtcgtaacagggtaaccg

SEQ ID NO: 4 - DNA, 1386 bp, HMI 4 Clostridium orbiscindens 16S rDNA
  source 1..1386: mol_type = genomic DNA
tggcggacgggtgagtaacgcgtgaggaacctgcctcggagtggggaataacagaccgaaaggcctgctaataccgcatgatgcagttggaccgcatggtcctgactgccaaagatttatcgctctgagatggcctcgcgtctgattagcttgttggcggggtaatggcccaccaaggcgacgatcagtagccggactgagaggttggccggccacattgggactgagacacggcccagactcctacgggaggcagcagtggggaatattgggcaatgggcgcaagcctgacccagcaacgccgcgtgaaggaagaaggctttcgggttgtaaacttcttttctcagggacgaacaaatgacggtacctgaggaataagccacggctaactacgtgccagcagccgcggtaatacgtaggtggcaagcgttatccggatttactgggtgtaaagggcgtgtaggcgggaaggcaagtcagatgtgaaaactatgggctcaacccatagcctgcatttgaaactgtttttcttgagtgctggagaggcaatcggaattccgtgtgtagcggtgaaatgcgtagatatacggaggaacaccagtggcgaaggcggattgctggacagtaactgacgctgaggcgcgaaagcgtggggagcaaacaggattagataccctggtagtccacgctgtaaacgatggatactaggtgtggggggtctgaccccctccgtgccgcagttaacacaataagtatcccacctggggagtacgatcgcaaggttgaaactcaaaggaattgacgggggcccgcacaagcggtggagtatgtggtttaattcgaagcaacgcgaagaaccttaccagggcttgacatcctactaacgaagcagagatgcattaggtgcccttcggggaaagtagagacaggtggtgcatggttgtcgtcagctcgtgtcgtgagatgttgggttaagtcccgcaacgagcgcaacccttattgttagttgctacgcaagagcactctagcgagactgccgttgacaaaacggaggaaggcggggacgacgtcaaatcatcatgccccttatgtcctgggctacacacgtactacaatggtggtaaacagagggaagcaagaccgcgaggtggagcaaatccctaaaagccatcccagttcggattgcaggctgaaacccgcctgtatgaagttggaatcgctagtaatcgcggatcagcatgccgcggtgaatacgttcccgggccttgtacacaccgcccgtcacaccatgagagtcgggaacacccgaagtccgtagtctaaccgcaagggggacgcggccgaaggtgggttcgataattggggtgaagtcgtaacagggtaacc

SEQ ID NO: 5 - DNA, 1324 bp, HMI 5 Ruminococcus flavefaciens 16S rDNA
  source 1..1324: mol_type = genomic DNA
cggatcagtggcggacgggtgagtaacacgtgagcaacctgcctttaagagggggataacgtttggaaacgaacgctaataccgcataacatagaagattcacatgtttcttctatcaaagatttatcgcttaaagatgggctcgcgtctgattagctagttggtgaggtaacggctcaccaaggcgacgatcagtagccgtactgagaggtagaacggccacattgggactgagacacggcccagactcctacgggaggcagcagtggggaatattgcacaatggaggaaactctgatgcagcgatgccgcgtgagggaagaaggttttcggattgtaaacctctgtcttcagggacgataatgacggtacctgaggaggaagctccggctaactacgtgccagcagccgcggtaatacgtagggagcgagcgttgtccggaattactgggtgtaaagggagcgtaggcgggatcttaagtcaggtgtgaaaactatgggctcaacccatagactgcacttgaaactgaggttcttgagtgaagtagaggcaggcggaattcctagtgtagcggtgaaatgcgtagatattaggaggaacatcagtggcgaaggcggcctgctgggcttttactgacgctgaggctcgaaagcgtggggagcaaacaggattagataccctggtagtccacgctgtaaacgatgattactaggtgtggggggactgaccccttccgtgccgcagttaacacaataagtaatccacctggggagtacggccgcaaggttgaaactcaaaggaattgacgggggcccgcacaagcagtggagtatgtggtttaattcgaagcacgcgaagaaccttaccgggtcttgacatctacagaatcctttagagataagggagtgcccttcggggaactgtaagacaggtggtgcatggttgtcgtcagctcgtgtcgtgagatgttgggttaagtcccgcaacgagcgcaacccctatcattagttgctacgcaagagcactctaatgagactgccgttgacaaaacggaggaaggtggggatgacgtcaaatcatcatgccccttatgacccgggctacacacgtactacaatggcgtaacagagggaagcaacatcgcgaggtgaagcaaatctctaaaaaacgtcccagttcagattgcaggctgcaactcgcctgcatgaagacggaattgctagtaatcgcagatcagcatgctgcggtgaatacgttcccgggccttgtacacaccgcccgtcacaccatgggagtcggtaacacccgaagtcgcttgtctaa

SEQ ID NO: 6 - DNA, 1426 bp, HMI 6 Anaerotruncus colihominis 16S rDNA
  source 1..1426: mol_type = genomic DNA
agtcgacggacacatccgacggaatagcttgctaggaagatggatgttgttagtggcggacgggtgagtaacacgtgagcaacctacctcagagtgggggacaacagttggaaacgactgctaataccgcataagatggcagggtcgcatggcctggtcataaaaggagcaattcgctctgagatgggctcgcgtctgattagctagttggtgaggtaacggctcaccaaggcaacgatcagtagccggactgagaggttgaacggccacattgggactgagacacggcccagactcctacgggaggcagcagtggggaatattgcacaatgggggaaaccctgatgcagcgacgccgcgtgagggaagacggttttcggattgtaaacctctgtcttgtgggacgatagtgacggtaccacaggaggaagccatggctaactacgtgccagcagccgcggtaatacgtagatggcgagcgttgtccggaattactgggtgtaaagggagtgtaggcgggctggtaagttgaatgtgaaaccttcgggctcaacccggagcgtgcgttcaaaactgctggtcttgagtgaagtagaggcaggcggaattcccggtgtagcggtggaatgcgtagatatcgggaggaacaccagtggcgaaggcggcctgctgggcttttactgacgctgaggctcgaaagcatgggtagcaaacaggattagataccctggtagtccatgccgtaaacgatgattactaggtgtggggggattgaccccctccgtgccggagttaacacaataagtaatccacctggggagtacgaccgcaaggttgaaactcaaaggaattgacgggggcccgcacaagcagtggagtatgtggtttaattcgaagcaacgcgaaaaaccttaccaggtcttgacatccatcgccaggctaagagattagctgttccctccggggacgatgagacaggtggtgcatggttgtcgtcagctcgtgtcgtgagatgttgggttaagtcccgcaacgagcgcaacccttactattagttgctacgcaagagcactctaatgggactgccgttgacaaaacggaggaaggtggggatgacgtcaaatcatcatgccccttatgacctgggctacacacgtactacaatggccgttaacagagagcagcgataccgcgaggtggagcgaatctagaaaaacggtctcagttcggattgcaggctgaaactcgcctgcatgaagtcggaattgctagtaatcgcggatcagcatgccgcggtgaatacgttcccgggccttgtacacaccgcccgtcacaccatgagagccggtaacacccgaagtcagtagcctaaccgcaaggagggcgctgccgaaggtggggctggtaattggggtgaagtcgtaac

SEQ ID NO: 7 - DNA, 1373 bp, HMI 7 Clostridium xylanolyticum 16S rDNA
  source 1..1373: mol_type = genomic DNA
gtaacgcgtgggtaacctgcctcatacagggggataacagttagaaatgactgctaataccgcataagcgcacagggtcgcatgacctagtgtgaaaaactccggtggtatgagatggacccgcgtctgattagctagttggtgaggtaacggctcaccaaggcgacgatcagtagccgacctgagagggtgatcggccacattgggactgagacacggcccaaactcctacgggaggcagcagtggggaatattgcacaatgggggaaaccctgatgcagcgacgccgcgtgaaggaagaagtatttcggtatgtaaacttctatcagcagggaagaaaatgacggtacctgactaagaagccccggctaactacgtgccagcagccgcggtaatacgtagggggcaagcgttatccggatttactgggtgtaaagggagcgtaggcggtctgacaagtcagaagtgaaagcccggggctcaactccgggactgcttttgaaactgccggactagattgcaggagaggtaagtggaattcctagtgtagcggtgaaatgcgtagatattaggaggaacaccagtggcgaaggcggcttactggactgtaaatgacgctgaggctcgaaagcgtggggagcaaacaggattagataccctggtagtccacgccgtaaacgatgaatactaggtgttggggagcacagctcttcggtgccgcagcaaacgcaataagtattccacctggggagtacgttcgcaagaatgaaactcaaaggaattgacggggacccgcacaagcggtggagcatgtggtttaattcgaagcaacgcgaagaaccttaccaagtcttgacatcccgatgaccgtcccgtaacgggggcttctcttcggagcatcggtgacaggtggtgcatggttgtcgtcagctcgtgtcgtgagatgttgggttaagtcccgcaacgagcgcaacccttatctttagtagccagcggtacggccgggcactctagagagactgccagggataacctggaggaaggtggggatgacgtcaaatcatcatgccccttatgatttgggctacacacgtgctacaatggcgtaaacaaagggaagcgaaactgtgaagtctagcaaatctcaaaaataacgtctcagttcggattgtagtctgcaactcgactacatgaagctggaatcgctagtaatcgcgaatcagcatgtcgcggtgaatacgttcccgggtcttgtacacaccgcccgtcacaccatgggagttggaaacgcccgaagtcagtgacccaaccgtaaggagggagctgccgaaggcgggtctgataactggggtgaagtcgtaacaaggtaaccg

SEQ ID NO: 8 - DNA, 1416 bp, HMI 8 Clostridium oroticum 16S rDNA
  source 1..1416: mol_type = genomic DNA
ttttgattgatttcttcggaaagagagagactgtgactgagtggcggacgggtgagtaacgcgtgggtaacctgcctcatacagggggataacagttagaaatgactgctaataccgcataagcacacagcttcgcatgaagcagtgtgaaaaactccggtggtatgagatggacccgcgtctgattaggtagttggtggggtaacggcccaccaagccgacgatcagtagccgacctgagagggtgaccggccacattgggactgagacacggcccaaactcctacgggaggcagcagtggggaatattgcacaatgggggaaaccctgatgcagcgacgccgcgtgaaggatgaagtatttcggtatgtaaacttctatcagcagggaagaaaatgacggtacctgactaagaagccccggctaactacgtgccagcagccgcggtaatacgtagggggcaagcgttatccggatttactgggtgtaaagggagcgtagacggtaatgcaagtctggagtgaaaacccggggctcaaccccgggactgctttggaaactgtgtaactagagtgtcggagaggcaagtggaattcctagtgtagcggtgaaatgcgtagatattaggaggaacaccagtggcgaaggcggcttgctggacgatgactgacgttgaggctcgaaagcgtggggagcaaacaggattagataccctggtagtccacgccgtaaacgatgactactaggtgtcggtaagcaaagcttatcggtgccgcagcaaacgcaataagtagtccacctggggagtacgttcgcaagaatgaaactcaaaggaattgacggggacccgcacaagcggtggagcatgtggtttaattcgaagcaacgcgaagaaccttacctggtcttgacatccctctgacagctgagtaatgtcggttttctttcgggacagaggagacaggtggtgcatggttgtcgtcagctcgtgtcgtgagatgttgggttaagtcccgcaacgagcgcaacccctatcttcagtagccagcatatgagatgggcactctggagagactgccagggataacctggaggaaggtggggatgacgtcaaatcatcatgccccttatgatcagggctacacacgtgctacaatggcgtaaacaaagggaagcgagcctgcgagggggagcaaatcccaaaaataacgtctcagttcggattgtagtctgcaactcgactacatgaagctggaatcgctagtaatcgcgaatcagaatgtcgcggtgaatacgttcccgggtcttgtacacaccgcccgtcacaccatgggagtcagtaacgcccgaagtcagtgacccaacctttcaggagggagctgccgaaggcgggaccgataactggggtgaagtcgt

SEQ ID NO: 9 - DNA, 1427 bp, HMI 9 Eubacterium contortum 16S rDNA
  source 1..1427: mol_type = genomic DNA
cttaagtttgattcttcggatgaagacttttgtgactgagtggcggacgggtgagtaacgcgtgggtaacctgcctcatacaggtggataacagttagaaatgactgctaataccgcataagaccacagcaccgcatggtgcaggggtaaaaactccggtggtatgagatggacccgcgtctgattagctagttggtggggtaacggcctaccaaggcgacgatcagtagccgacctgagagggtgaccggccacattgggactgagacacggcccaaactcctacgggaggcagcagtggggaatattgcacaatgggggaaaccctgatgcagcgacgccgcgtgaaggatgaagtatttcggtatgtaaacttctatcagcagggaagaaaatgacggtacctgactaagaagccccggctaactacgtgccagcagccgcggtaatacgtagggggcaagcgttatccggatttactgggtgtaaagggagcgtagacggtatggcaagtctgatgtgaaaggccagggctcaaccctgggactgcattggaaactgtcgaactagagtgtcggagaggcaagtggaattcctagtgtagcggtgaaatgcgtagatattaggaggaacaccagtggcgaaggcggcttgctggacgatgactgacgttgaggctcgaaagcgtggggagcaaacaggattagataccctggtagtccacgccgtaaacgatgactactaggtgtcgggtagcagagctattcggtgccgcagccaacgcaataagtagtccacctggggagtacgttcgcaagaatgaaactcaaaggaattgacggggacccgcacaagcggtggagcatgtggtttaattcgaagcaacgcgaagaaccttacctgctcttgacatctccctgaccggcaagtaatgttgcctttccttcgggacagggatgacaggtggtgcatggttgtcgtcagctcgtgtcgtgagatgttgggttaagtcccgcaacgagcgcaacccctatctttagtagccagcggtttggccgggcactctagagagactgccagggataacctggaggaaggtggggatgacgtcaaatcatcatgccccttatgagcagggctacacacgtgctacaatggcgtaaacaaagggaagcgagcctgcgagggtaagcaaatctcaaaaataacgtctcagttcggattgtagtctgcaactcgactacatgaagctggaatcgctagtaatcgcgaatcagaatgtcgcggtgaatacgttcccgggtcttgtacacaccgcccgtcacaccatgggagttggtaacgcccgaagtcagtgacccaaccgcaaggagggagctgccgaaggtgggaccgataactggggtgaagtcgtaacaaggtaaccg

SEQ ID NO: 10 - DNA, 1447 bp, HMI 10 Clostridium oroticum 16S rDNA
  source 1..1447: mol_type = genomic DNA
acatgcaagtcgagcgagcgctttagtggaattctacggaaggaaagtgaagtgactgagcggcggacgggtgagtaacgcgtgggtaacctgcctcatacagggggataacagttagaaatgactgctaataccgcataagaccccagtaccgcatggtacagaggtaaaaactgaggtggtatgagatggacccgcgtctgattagctagttggtgaggtagaggctcaccaaggcgacgatcagtagccgacctgagagggtgaccggccacattgggactgagacacggcccaaactcctacgggaggcagcagtggggaatattgcacaatgggggaaaccctgatgcagcgacgccgcgtgagcgaagaagtatttcggtatgtaaagctctatcagcagggaagaaaatgacggtacctgactaagaagcaccggctaaatacgtgccagcagccgcggtaatacgtatggtgcaagcgttatccggatttactgggtgtaaagggagcgtagacggagcagcaagtctgatgtgaaaacccggggctcaaccccgggagtgcattggaaactgttgatctagagtgctggagaggtaagtggaattcctagtgtagcggtgaaatgcgtagatattaggaggaacaccagtggcgaaggcggcttactggacagtgactgacgttgaggctcgaaagcgtggggagcaaacaggattagataccctggtagtccacgccgtaaacgatgactactaggtgtcgggtagcaaagctattcggtgccgcagccaacgcaataagtagtccacctggggagtacgttcgcaagaatgaaactcaaaggaattgacggggacccgcacaagcggtggagcatgtggtttaattcgaagcaacgcgaagaaccttacctgcccttgacatccgggtgaccggcgagtaatgtcgccttctcttcggagcagccgagacaggtggtgcatggttgtcgtcagctcgtgtcgtgagatgttgggttaagtcccgcaacgagcgcaacccttatctttagtagccagcggataagccggggactctagagagactgccagggataacctggaggaaggtggggatgacgtcaaatcatcatgccccttatgggcagggctacacacgtgctacaatggcgtaaacaaagggaagcgaagctgtgaagcggagcgaatctcaaaaataacgtctcagttcggattgtagtctgcaactcgactacatgaagctggaatcgctagtaatcgcgaatcagaatgtcgcggtgaatacgttcccgggtcttgtacacaccgcccgtcacaccatgggagtcagtaacgcccgaagtcagtgacccaaccgtaaggagggagctgccgaaggcgggacggataactggggtgaagtcgtaacaaggtaaccg

SEQ ID NO: 11 - DNA, 1379 bp, HMI 11 Lachnospira pectinoschiza 16S rDNA
  source 1..1379: mol_type = genomic DNA
agtggcggacgggtgagtaacgcgtgggtaacctgccctgtacagggggacaacagctggaaacggctgctaataccgcataagcccttagcactgcatggtgcatagggaaaaggagcaatccggtacaggatggacccgcgtctgattagccagttggcagggtaacggcctaccaaagcgacgatcagtagccgatctgagaggatgtacggccacattgggactgagacacggcccagactcctacgggaggcagcagtggggaatattgcacaatggaggaaactctgatgcagcgacgccgcgtgagtgaagaagtatttcggtatgtaaagctctatcagcagggaagaaaatgacggtacctgactaagaagcaccggctaaatacgtgccagcagccgcggtaatacgtatggtgcaagcgttatccggatttactgggtgtaaagggagcgtaggtggcaaggcaagccagaagtgaaaacccggggctcaaccgcgggattgcttttggaactgtcatgctagagtgcaggaggggtgagcggaattcctagtgtagcggtgaaatgcgtagatattaggaggaacaccggaggcgaaggcggctcactggactgtaactgacactgaggctcgaaagcgtggggagcaaacaggattagataccctggtagtccacgcggtaaacgatgaatactagatgtcgggtagcaaagctactcggtgtcgtcgcaaacgcaataagtattccacctggggagtacgttcgcaagaatgaaactcaaaggaattgacggggacccgcacaagcggtggagcatgtggtttaattcgaagcaacgcgaagaaccttacctgctcttgacatcccattcgatagagggtaatgcttctagcccttcgggggaatggagacaggtggtgcatggttgtcgtcagctcgtgtcgtgagatgttgggttaagtcccgcaacgagcgcaacccttattgtcagtagccagcaggtgaagctgggcactctgatgagactgccggggataacccggaggaaggtggggatgacgtcaaatcatcatgccccttatgagcagggctacacacgtgctacaatggcgtaaacagagggaagcgaaggagtgatctggagcaaatctcaaaaataacgtctcagttcggattgtagtctgcaactcgactacatgaagctggaatcgctagtaatcgcagatcaaaatgctgcggtgaatacgttcccgggtcttgtacacaccgcccgtcacaccatgggagtcggtaatgcccgaagtcagtgactcaaccgaaaggaaaaagctgccgaaggcaggactggtaactggggtgaagtcgt

SEQ ID NO: 12 - DNA, 1444 bp, HMI 12 Roseburia faecis 16S rDNA
  source 1..1444: mol_type = genomic DNA
agtcgaacgaagcactttattacgatttcttcggaatgacgatttagtgactgagtggcggacgggtgagtaacgcgtgggtaacctgccttatacagggggataacagttagaaatgactgctaataccgcataagcgcacaggattgcatgatctggtgtgaaaaactccggtggtataagatggacccgcgtctgattagctggttggtgaggtaacggcccaccaaggcgacgatcagtagccgacctgagagggtgaccggccacattgggactgagacacggcccaaactcctacgggaggcagcagtggggaatattgcacaatgggggaaaccctgatgcagcgacgccgcgtgagcgaagaagtatttcggtatgtaaagctctatcagcagggaagaaaaaaatgacggtacctgactaagaagccccggctaactacgtgccagcagccgcggtaatacgtagggggcaagcgttatccggatttactgggtgtaaagggagcgcaggcggtgcggcaagtctgatgtgaaagcccggggctcaaccccgggactgcattggaaactgtcgtacttgagtatcggagaggtaagtggaattcctagtgtagcggtgaaatgcgtagatattaggaggaacaccagtggcgaaggcggcttactggacgataactgacgctgaggctcgaaagcgtggggagcaaacaggattagataccctggtagtccacgccgtaaacgatgaatactaggtgtcgggggacatagtccttcggtgccgcagcaaacgcaataagtattccacctggggagtacgttcgcaagaatgaaactcaaaggaattgacggggacccgcacaagcggtggagcatgtggtttaattcgaagcaacgcgaagaaccttaccaagtcttgacatcccggtgacaaagtatgtaatgtactctttcttcggaacaccggtgacaggtggtgcatggttgtcgtcagctcgtgtcgtgagatgttgggttaagtcccgcaacgagcgcaacccctgttcttagtagccagcggttcggccgggcactctagggagactgccagggataacctggaggaaggcggggatgacgtcaaatcatcatgccccttatgacttgggctacacacgtgctacaatggcgtaaacaaagggaagcgaaaaggtgacttctagcaaatcccaaaaataacgtcccagttcggactgtagtctgcaactcgactacacgaagctggaatcgctagtaatcgcgaatcagaatgtcgcggtgaatacgttcccgggtcttgtacacaccgcccgtcacaccatgggagtcgggaatgcccgaagccggtgactcaaccgaaaggagagagccgtcgaaggcaggtctgataactggggtgaagtcgtaacaaggtaacc

SEQ ID NO: 13 - DNA, 1452 bp, HMI 14 Clostridium hathewayi 16S rDNA
  source 1..1452: mol_type = genomic DNA
agtcgacggagatgcgatgtgagcgagaggtgcttgcactgatcaatcttttcgtatcttagtggcggacgggtgagtaacgcgtgggtaacctgccttataccgggggataacacttagaaataggtgctaataccgcataagcgcacggtgtcgcatgacacagtgtgaaaaactccggtggtataagatggacccgcgtctgattagccagttggcagggtaacggcctaccaaagcgacgatcagtagccggcctgagagggtgaacggccacattgggactgagacacggcccaaactcctacgggaggcagcagtggggaatattgcacaatgggggaaaccctgatgcagcgacgccgcgtgagtgaagaagtatttcggtatgtaaagctctatcagcagggaagaagaaatgacggtacctgactaagaagccccggctaactacgtgccagcagccgcggtaatacgtagggggcaagcgttatccggatttactgggtgtaaagggagcgtagacggtgaagcaagtctgaagtgaaaggttggggctcaaccccgaaactgctttggaaactgtttaactggagtacaggagaggtaagtggaattcctagtgtagcggtgaaatgcgtagatattaggaggaacaccagtggcgaaggcggcttactggactgtaactgacgttgaggctcgaaagcgtggggagcaaacaggattagataccctggtagtccacgccgtaaacgatgattactaggtgttggtggatatggatccatcggtgccgcagcaaacgcaataagtaatccacctggggagtacgttcgcaagaatgaaactcaaaggaattgacggggacccgcacaagcggtggagcatgtggtttaattcgaagcaacgcgaagaaccttacctgatcttgacatccctatgaatacagggtaatgcctgtagtacttcggtacataggagacaggtggtgcatggttgtcgtcagctcgtgtcgtgagatgttgggttaagtcccgcaacgagcgcaacccctatctttagtagccagcagtaagatgggcactctagagagactgccggggataacccggaggaaggtggggatgacgtcaaatcatcatgccccttatgaccagggctacacacgtgctacaatggcgtaaacagagggaagcgaagtggtgacatggagcaaatcccaaaaataacgtcccagttcggattgcaggctgcaactcgcctgcatgaagctggaatcgctagtaatcgcagatcagaatgctgcggtgaatacgttcccgggtcttgtacacaccgcccgtcacaccatgggagtaggtaatgcccgaagtcggtgacctaaccgcaaggaaggagccgccgaaggcaggacttataactggggtgaagtcgtaacaaggtaaccgt

SEQ ID NO: 14 - DNA, 1400 bp, HMI 15 Fusicatenibacter saccharivorans 16S rDNA
  source 1..1400: mol_type = genomic DNA
cggatggaatcggtataacttagtggcggacgggtgagtaacgcgtgggaaacctgccctgtaccgggggataacacttagaaataggtgctaataccgcataagcgcacggaactgcatggttctgtgtgaaaaactccggtggtacaggatggtcccgcgtctgattagccagttggcagggtaacggcctaccaaagcgacgatcagtagccggcctgagagggtgaacggccacattgggactgagacacggcccaaactcctacgggaggcagcagtggggaatattgcacaatgggggaaaccctgatgcagcgacgccgcgtgagtgaagaagtatttcggtatgtaaagctctatcagcagggaagaaaatgacggtacctgactaagaagccccggctaactacgtgccagcagccgcggtaatacgtagggggcaagcgttatccggatttactgggtgtaaagggagcgtagacggcatggcaagccagatgtgaaaacccagggctcaaccttgggattgcatttggaactgccaggctggagtgcaggagaggtaagcggaattcctagtgtagcggtgaaatgcgtagatattaggaggaacaccagtggcgaaggcggcttactggactgtaactgacgttgaggctcgaaagcgtggggagcaaacaggattagataccctggtagtccacgcggtaaacgatgattgctaggtgtaggtgggtatggacccatcggtgccgcagctaacgcaataagcaatccacctggggagtacgttcgcaagaatgaaactcaaaggaattgacggggacccgcacaagcggtggagcatgtggtttaattcgaagcaacgcgaagaaccttaccaagtcttgacatcccaatgacgcacctgtaaagaggtgttcccttcggggcattggagacaggtggtgcatggttgtcgtcagctcgtgtcgtgagatgttgggttaagtcccgcaacgagcgcaacccttattcttagtagccagcaggtgaagctgggcactctaaggagactgccggggataacccggaggaaggcggggatgacgtcaaatcatcatgccccttatgatttgggctacacacgtgctacaatggcgtaaacaaagggaagcgagacagtgatgtggagcaaatcccagaaataacgtctcagttcggattgtagtctgcaactcgactacatgaagctggaatcgctagtaatcgcgaatcagcatgtcgcggtgaatacgttcccgggtcttgtacacaccgcccgtcacaccatgggagttggaaatgcccgaagtctgtgacctaaccgaaagggaggagcagccgaaggcaggtctgataactggggtgaagtcgta

SEQ ID NO: 15 - DNA, 1416 bp, HMI 16 Clostridium clostridioforme 16S rDNA
  source 1..1416: mol_type = genomic DNA
ctgctttgatgaagttttcggatggatttaaaacagcttagtggcggacgggtgagtaacgcgtgggtaacctgcctcacactgggggataacagttagaaatagctgctaataccgcataagcgcacggttccgcatggaacagtgtgaaaaactccggtggtgtgagatggacccgcgtctgattagccagttggcggggtaacggcccaccaaagcgacgatcagtagccggcctgagagggtgaacggccacattgggactgagacacggcccaaactcctacgggaggcagcagtggggaatattgcacaatgggggaaaccctgatgcagcgacgccgcgtgagtgaagaagtatttcggtatgtaaagctctatcagcagggaagaaagtgacggtacctgaataagaagccccggctaactacgtgccagcagccgcggtaatacgtagggggcaagcgttatccggatttactgggtgtaaagggagcgtagacggcaaggcaagtctgaagtgaaagcccggtgcttaacgccgggactgctttggaaactgtttagctggagtgccggagaggtaagcggaattcctagtgtagcggtgaaatgcgtagatattaggaagaacaccagtggcgaaggcggcttactggacggtaactgacgttgaggctcgaaagcgtggggagcaaacaggattagataccctggtagtccacgccgtaaacgatgattgctaggtgtaggtgggtatggacccatcggtgccgcagctaacgcaataagcaatccacctggggagtacgttcgcaagaatgaaactcaaaggaattgacggggacccgcacaagcggtggagcatgtggtttaattcgaagcaacgcgaagaaccttaccaggtcttgacatcccgatgaaaaacccgtaacggggttccctcttcggagcatcggagacaggtggtgcatggttgtcgtcagctcgtgtcgtgagatgttgggttaagtcccgcaacgagcgcaacccttattcttagtagccagcaggtaaggctgggcactctaaggagactgccggggataacccggaggaaggtggggatgacgtcaaatcatcatgccccttatgatctgggctacacacgtgctacaatggcgtaacaaagggaagcgagcctgcgagggtgagcaaatcccaaaaataacgtcccagttcggactgtagtctgcaacccgactacacgaagctggaatcgctagtaatcgcgaatcagaatgtcgcggtgaatacgttcccgggtcttgtacacaccgcccgtcacaccatgggagtcggaaatgcccgaagtctgtgactcaaccgcaaggagagagcagccgaaggcaggtctgataactggggtgaagtcgt

SEQ ID NO: 16 - DNA, 1211 bp, HMI 17 Rumincoccus torques 16S rDNA
  source 1..1211: mol_type = genomic DNA
cggtatgagatggacccgcgtctgattagctagttggtggggtaacggcctaccaaggcgacgatcagtagccgacctgagagggtgaccggccacattgggactgagacacggcccaaactcctacgggaggcagcagtggggaatattgcacaatgggggaaaccctgatgcagcgacgccgcgtgagcgaagaagtatttcggtatgtaaagctctatcagcagggaagaaaatgacggtacctgactaagaagccccggctaactacgtgccagcagccgcggtaatacgtagggggcaagcgttatccggatttactgggtgtaaagggagcgtagacggcgaggcaagtctgatgtgaaaacccggggctcaaccccgtgactgcattggaaactgttttgcttgagtgccggagaggtaagcggaattcctagtgtagcggtgaaatgcgtagatattaggaggaacaccagtggcgaaggcggcttactggacggcaactgacgttgaggctcgaaagcgtggggagcaaacaggattagataccctggtagtccacgccgtaaacgatgaatactaggtgtcggggagcaaagctcttcggtgccgccgcaaacgcaataagtattccacctggggagtacgttcgcaagaatgaaactcaaaggaattgacggggacccgcacaagcggtggagcatgtggtttaattcgaagcaacgcgaagaaccttaccaagccttgacatcccattgacagagcatgtaatgtgctttcccttcggggcagtggtgacaggtggtgcatggttgtcgtcagctcgtgtcgtgagatgttgggttaagtcccgcaacgagcgcaacccctatcttcagtagccagcggtttggccgggcactctggagagactgccagggataacctggaggaaggtggggatgacgtcaaatcatcatgccccttatggcttgggctacacacgtgctacaatggcgtaaacaaagggaagcgagcctgcgagggggagcaaatcccaaaaataacgtctcagttcggattgtagtctgcaactcgactacatgaagctggaatcgctagtaatcgcgaatcagaatgtcgcggtgaatacgttcccgggtcttgtacacaccgcccgtcacaccatgggagtcggcaacgcccgaagccagtgacccaaccgaaag

SEQ ID NO: 17 - DNA, 1425 bp, HMI 18 Closstridium celerecrescens 16S rDNA
  source 1..1425: mol_type = genomic DNA
agtcgacgaggtaatgagatgaagttttcggatggattcttatttccgagtggcggacgggtgagtaacgcgtgggtaacctgcctcatacagggggataacgattggaaacgattgctaataccgcataagcgcacagtaccacatggtacagtgtgaaaaactccggtggtatgagatggacccgcgtctgattagctagttggtgaggtaacggcccaccaaggcaacgatcagtagccgacctgagagggtgaccggccacattgggactgagacacggcccagactcctacgggaggcagcagtgggggatattgcacaatggaggaaactctgatgcagcgacgccgcgtgagtgaagaagtatttcggtatgtaaagctctatcagcagggaagaaaatgacggtacctgactaagaagccccggctaactacgtgccagcagccgcggtaatacgtagggggcaagcgttatccggatttactgggtgtaaagggagcgtagacggcgatgcaagtctgaagtgaaatacccgggctcaacctgggaactgctttggaaactgtatggctagagtgctggagaggtaagcggaattcctagtgtagcggtgaaatgcgtagatattaggaagaacaccagtggcgaaggcggcttactggacagtaactgacgttcaggctcgaaagcgtggggagcaaacaggattagataccctggtagtccacgccgtaaacgatgaatactaggtgtcgggggacaaagtctttcggtgccgccgcaaacgcaataagtattccacctggggagtacgttcgcaagaatgaaactcaaaggaattgacggggacccgcacaagcggtggagcatgtggtttaattcgaagcaacgcgaagaaccttaccaaatcttgacatccctctgaaaagcctttaatcgagctcctccttcgggacagaggtgacaggtggtgcatggttgtcgtcagctcgtgtcgtgagatgttgggttaagtcccgcaacgagcgcaacccctattgtcagtagccagcaggtaaagctgggcactctgatgagactgccagggataacctggaggaaggtggggatgacgtcaaatcatcatgccccttatgatttgggctacacacgtgctacaatggcgtaaacaaagagaggcgaagctgtgaggcagagcaaatctcaaaaataacgtctcagttcggattgtagtctgcaactcgactacatgaagctggaatcgctagtaatcgcggatcagaatgccgcggtgaatacgttcccgggtcttgtacacaccgcccgtcacaccatgggagtcggaaatgcccgaagccagtgacccaagcgaaagcagggagctgtcgaaggcaggtctgataactggggtgaagtcgt

SEQ ID NO: 18 - DNA, 1437 bp, HMI 19 Clostridium celerescens 16S rDNA
  source 1..1437: mol_type = genomic DNA
tcgacgaggtattttgattgaagttttcggatggatttcagataccgagtggcggacgggtgagtaacgcgtgggtaacctgcctcatacagggggataacggttagaaatgactgctaataccgcataagcgcacagtaccgcatggtacggtgtgaaaaactccggtggtatgagatggacccgcgtctgattagctagttggtggggtaacggcccaccaaggcgacgatcagtagccgacctgagagggtgaccggccacattgggactgagacacggcccagactcctacgggaggcagcagtgggggatattgcacaatggaggaaactctgatgcagcgacgccgcgtgagtgaagaagtatttcggtatgtaaagctctatcagcagggaagaaaatgacggtacctgactaagaagccccggctaactacgtgccagcagccgcggtaatacgtagggggcaagcgttatccggatttactgggtgtaaagggagcgtagacggcgacgcaagtctgaagtgaaatacccgggctcaacctgggaactgctttggaaactgtgttgctagagtgctggagaggtaagcggaattcctagtgtagcggtgaaatgcgtagatattaggaagaacaccagtggcgaaggcggcttactggacagtaactgacgttgaggctcgaaagcgtggggagcaaacaggattagataccctggtagtccacgccgtaaacgatgaatactaggtgttggtgagcaaagctcatcggtgccgccgcaaacgcaataagtattccacctggggagtacgttcgcaagaatgaaactcaaaggaattgacggggacccgcacaagcggtggagcatgtggtttaattcgaagcaacgcgaagaaccttaccaaatcttgacatccctctgaaacgcccttaatcgggctcctccttcgggacagaggtgacaggtggtgcatggttgtcgtcagctcgtgtcgtgagatgttgggttaagtcccgcaacgagcgcaacccctattgtcagtagccagcaggtaaagctgggcactctgatgagactgccagggataacctggaggaaggtggggatgacgtcaaatcatcatgccccttatgatttgggctacacacgtgctacaatggcgtaaacaaagagaagcgagcctgcgagggggagcaaatctcaaaaataacgtctcagttcggattgtagtctgcaactcgactacatgaagctggaatcgctagtaatcgcagatcagaatgctgcggtgaatacgttcccgggtcttgtacacaccgcccgtcacaccatgggagtcggaaatgcccgaagccagtgacccaagcgaaagcagggagctgtcgaaggcaggtctgataactggggtgaagtcgtaacagggtaaccg

SEQ ID NO: 19 - DNA, 1401 bp, HMI 20 Eubacterium infirmum 16S rDNA
  source 1..1401: mol_type = genomic DNA
gagctcatcacagatgcttcggttgaagtgatgagtggaaagcggcggacgggtgagtaacgcgtaggcaacctgccctttgcagagggatagcctcgggaaaccgggattaaaacctcatgacacctcttaaagacatctttgagaggtcaaagatttatcggcagaggatgggcctgcgtctgattagctagttggtggggtaacggcctaccaaggcgacgatcagtagccgacctgagagggtgatcggccacattggaactgagacacggtccaaactcctacgggaggcagcagtggggaatattgcacaatgggggaaaccctgatgcagcaacgccgcgtgaaggaagaaggcctttgggtcgtaaacttctgttctaagggaagataatgacggtaccttaggagcaagtcccggctaactacgtgccagcagccgcggtaatacgtagggggcaagcgttatccggaattattgggcgtaaagagtacgtaggtggttacctaagcacgaggtataaggcaatggcttaaccattgttcgccttgtgaactgggctacttgagtgcaggagaggaaagcggaattcctagtgtagcggtgaaatgcgtagatattaggaggaacaccagtggcgaaggcggctttctggactgtaactgacactgaggtacgaaagcgtggggagcaaacaggattagataccctggtagtccacgccgtaaacgatgagcactaggtgtcggggtcgcaagacttcggtgccgcagttaacgcaataagtgctccgcctggggagtacgttcgcaagaatgaaactcaaaggaattgacggggacccgcacaagcagcggagcatgtggtttaattcgaagcaacgcgaagaaccttaccaggacttgacatccctctgacagccttttaatcgaggttttctacggacagaggagacaggtggtgcatggttgtcgtcagctcgtgtcgtgagatgttgggttaagtcccgcaacgagcgcaacccttgtcattagttgccagcagtaagatgggcactctagtgagactgccggggataactcggaggaaggtggggatgacgtcaaatcatcatgccccttatgttctgggctacacacgtgctacaatggccggtacagagagaaagcgagactgcgaagtggagcgaaactcaaaagccggtcccagttcggattgcaggctgcaactcgcctgcatgaagtcggagttgctagtaatcgcagatcagaatgctgcggtgaatgcgttcccgggtcttgtacacaccgcccgtcacaccatggaagttgggggcgcccgaagttggcagataaatatgttacctaaggcgaaatcaatgactggggtgaagtcgt

SEQ ID NO: 20 - DNA, 1368 bp, HMI 21 Eubacterium infirmum 16S rDNA
  source 1..1368: mol_type = genomic DNA
tcggtaaagggatatggcggaaagcggcggacgggtgagtaacgcgtaggcaacctgccccttacagagggatagccattggaaacgatgattaagacctcataacgcctccctcccacatgagggggaggccaaagattcatcggtaagggatgggcctgcgtctgattagcttgttggcggggtaacggcccaccaaggcgacgatcagtagccgacctgagagggtgatcggccacattggaactgagacacggtccaaactcctacgggaggcagcagtggggaatattgcacaatgggcggaagcctgatgcagcaacgccgcgtgagggatgaaggccttcgggtcgtaaacctctgtccttggggaagaaacaaatgacggtacccatggaggaagccccggctaactacgtgccagcagccgcggtaatacgtagggggcgagcgttatccggaattattgggcgtaaagagtgcgtaggtggttacctaagcgcagggtctaaggcaatggctcaaccattgttcgccctgcgaactgggctacttgagtgcaggagaggaaagcggaattcctagtgtagcggtgaaatgcgtagatattaggaggaacaccagtggcgaaggcggctttctggactgttactgacactgaggcacgaaagcgtggggagcaaacaggattagataccctggtagtccacgccgtaaacgatgagcactaggtgtcggggccgcaaggcttcggtgccgcagttaacgcattaagtgctccgcctggggagtacgcacgcaagtgtgaaactcaaaggaattgacggggacccgcacaagcagcggagcatgtggtttaattcgaagcaacgcgaagaaccttaccaggacttgacatccccctgacagatccttaaccggatccttcttcggacaggggagacaggtggtgcatggttgtcgtcagctcgtgtcgtgagatgttgggttaagtcccgcaacgagcgcaacccttgccattagttgccatcattcagttgggcactctaatgggactgccggggacaactcggaggaaggtggggatgacgtcaaatcatcatgccccttatgttctgggctacacacgtgctacaatggccggtacagcaggaagcgatcccgcgagggggagcaaatcccaaaaaccggtcccagttcggactgcaggctgcaacccgcctgcacgaagccggagttgctagtaatcgtggatcagaatgccacggtgaatgcgttcccgggtcttgtacacaccgcccgtcacaccatggaagttgggggtgcccgaagccggcagggagatatgctgtctaaggcaaaaccaat

SEQ ID NO: 21 - DNA, 1421 bp, HMI 22 Clostridium thermocellum 16S rDNA
  source 1..1421: mol_type = genomic DNA
ggatgaggaaatgcttcggcatggagacatccgatctagtggcggacgggtgagtaacgcgtgagcaacctgtcctgcacagggggataacactgagaaatcagtgctaataccgcatgagaccacagtatcacatggtacaggggtcaaaggagaaatccggtgcagggtgggctcgcgtcccattagctagttggtagggtaaaggcctaccaaggcgacgatgggtagccggactgagaggttggccggccacactgggactgagacacggcccagactcctacgggaggcagcagtggggaatattgggcaatgggcgaaagcctgacccagcaacgccgcgtgaaggaagaaggtctttggattgtaaacttttgtcctatgggaagaaggaagtgacggtaccatgggaggaagccccggctaactacgtgccagcagccgcggtaatacgtagggggcgagcgttgtccggaattactgggcgtaaagggcgcgcaggcggccgatcaagttagatgtgaaatacccgggcttaacctgggaactgcatttaaaactggttggctaggagtgcaggagagggaagcggaattcctagtgtagcggtgaaatgcgtagatattaggaggaacaccagtggcgaaggcggctttctggactgtaactgacgctgaggcgcgaaagcgtggggagcgaacaggattagataccctggtagtccacgctgtaaacgatgaatactaggtgtagggggtatcgaccccccctgtgccggagcaaacgcaataagtattccgcctggggagtacggccgcaaggttgaaactcaaaggaattgacgggggcccgcacaagcagcggagcatgtggtttaattcgaagcaacgcgaagaaccttaccaggtcttgacatccctcgaagtgcatagagatatgtacgtccttcgggacgaggagacaggtggtgcatggttgtcgtcagctcgtgtcgtgagatgttgggttaagtcccgcaacgagcgcaacccctacagttagttaccagcgggtaaagccggggactctaacaggactgccgtggataacacggaggaaggtggggacgacgtcaaatcatcatgctccttatgacctgggctacacacgtgctacaatggccggtacaaagagaagcgagaccgtaaggtggagcggatctcaaaaaaccggtcccagttcggattgtgggctgcaacccgcccacatgaagttggagttgctagtaatcgcgaatcagcatgtcgcggtgaatgcgttcccgggccttgtacacaccgcccgtcacaccatgggagttgggagcgcccgaagtcgttgaggtaacccgcaagggagccaggcgccgaaggtgagaccgataactggggtgaagtcgt

SEQ ID NO: 22 - DNA, 1507 bp, HMI 23 Anaerovorax odorimutans 16S rDNA
  source 1..1507: mol_type = genomic DNA
agagtttgatcctggctcaggatgaacgctggcggcgtgcctaacacatgcaagtcgagcgggaaatcttggaacgatacttcggtaaagggaagagatggatagcggcggacgggtgagtaacgcgtaggtaacctgcctcatgcagagggatagcctcgggaaactgggattaatacctcataatgcggaggagtcacatggctccatcgccaaagatttatcggcatgagatggacctgcgtctgattagttagttggtgaggtaacggctcaccaaggcagcgatcagtagccgacctgagagggtaatcggccacattggaactgagacacggtccaaactcctacgggaggcagcagtggggaatattgcacaatgggcgcaagcctgatgcagcaacgccgcgtgagcgatgaaggtcttcggatcgtaaagctctgtcctaggggaagaatatatgacggtacccttggaggaagccccggctaactacgtgccagcagccgcggtaatacgtagggggcgagcgttatccggaattattgggcgtaaagagttcgtaggtggttttgtaagcgcggggtttaaggcaacggctcaaccgttgttcgccttgcgaactgcaagacttgagtgcgggagaggaaagtggaattcctagtgtagcggtgaaatgcgtagatattaggaggaacaccagtggcgaaggcgactttctggaccgtaactgacactgaggaacgaaagcgtggggagcaaacaggattagataccctggtagtccacgccgtaaacgatgagcactaggtgtcggggccgcaaggtttcggtgccgcagttaacgcattaagtgctccgcctggggagtacgcacgcaagtgtgaaactcaaaggaattgacggggacccgcacaagcagcggagcatgtggtttaattcgaagcaacgcgaagaaccttaccagggcttgacatcccgatgaccggcgggtaacgccgccttctcttcggagcatcggtgacaggtggtgcatggttgtcgtcagctcgtgtcgtgagatgttgggttaagtcccgcaacgagcgcaacccttgtcattagttgccagcagttcggctgggcactctagtgagactgccggggacaactcggaggaaggtggggatgacgtcaaatcatcatgccccttatgttctgggctacacacgtgctacaatggccggtacagagagacgcaagactgtgaagtggagcaaaactctaaaaccggtcccagttcggattgtaggctgcaactcgcctacatgaagttggagttgctagtaatcgcgaatcagaatgtcgcggtgaatgcgttcccgggtcttgtacacaccgcccgtcacaccatggaagttgggggcgcccgaagttggtcaacaaatcgattacctaaggcgaaaccaatgactggggtgaagtcgtaacaaggtagccgtatcggaaggtgcggctggatcacct

SEQ ID NO: 23 - DNA, 1378 bp, HMI 24 Clostridium saccharogumia 16S rDNA
  source 1..1378: mol_type = genomic DNA
agccaccggcttcgggtgttatcaactctcatggtgtgacgggcggtgtgtacaaggcccgagaacgtattcaccgcggcatgctgatccgcgattactagcgattccatcttcatgcaggcgagttgcagcctgcaatccgaactgagaacgggtttttgagtttcgctccaagtcgcctcttcgcttccctttgatccgtccattgtagcacgtgtgtagcccaggtcataaggggcatgatgatttgacgtcatccccgccttcctccggcttgtcaccggctgtctcgttagagtccccatcttactgctggtaactaacgacaagggttgcgctcgttgcgggacttaacccaacatctcacgacacgagctgacgacaaccatgcaccacctgtcttgagtatatctatccctctatctctagagtctttactctgatgtcaagacctggtaaggttcttcgcgttgcttcgaattaaaccacatgctccaccgcttgtgcgggcccccgtcaattcctttgagtttcattcttgcgaacgtactactcaggcggagtacttattgcgttaactgcagcactgaggcttgtccccccaacacttagtactcatcgtttacggcgtggactactagggtatctaatcctatttgctccccacgctttcgggactgagcgtcagttacagaccagatcgtcgccttcgccactggtgttcctccatatatctacgcatttcaccgctacacatggaattccacgatcctcttctgcactctagctatttggtttccatggcttactgaagttaagcttcagccttttaccacagacctccattgccgcctgctccctctttacgcccaataattccggataacgcttgccacctacgtattaccgcggctgctggcacgtagttagccgtggcttcctcacaaagtaccgtcactctaataccattccctgtattagtcgttcttcctttataacagaagtttacaacccgaaggccttcttccttcacgcggcgttgctcggtcagggttccccccattgccgaaaattccctactgctgcctcccgtaggagtctgggccgtgtctcagtcccagtgtggccgttcaccctctcaggccggctatgcatcgtcgccttggtaggccgttacccctccaactagctaatgcaccataagcccatctgttccctatcccttaggatatttaacttagagaaaatgcttcctctaagcctatgcggtgttagcgcatgtttccacgcgttatccccctggtacagccaggttgcttatgtcttactcacccgttcgccactcatcaccgaagtgatgcgttcgacttgcatgtat

SEQ ID NO: 24 - DNA, 1376 bp, HMI 25 Clostridium saccharogumia 16S rDNA
  source 1..1376: mol_type = genomic DNA
ggcatctacagggggataactgatggaaacgtcagctaagaccgcataggtgtagagatcgcatgaactctatatgaaaagtgctacgggactggtagatgatggacttatggcgcattagcttgttggtagggtaacggcctaccaaggcgacgatgcgtagccgacctgagagggtgaccggccacactgggactgagacacggcccagactcctacgggaggcagcagtagggaattttcggcaatgggggaaaccctgaccgagcaacgccgcgtgaaggaagaagtaattcgttatgtaaacttctgtcatagaggaagaacggtggatatagggaatgatatccaagtgacggtactctataagaaagccacggctaactacgtgccagcagccgcggtaatacgtaggtggcgagcgttatccggaattattgggcgtaaagagggagcaggcggcactaagggtctgtggtgaaagatcgaagcttaacttcggtaagccatggaaaccgtagagctagagtgtgtgagaggatcgtggaattccatgtgtagcggtgaaatgcgtagatatatggaggaacaccagtggcgaaggcgacgatctggcgcataactgacgctcagtcccgaaagcgtggggagcaaataggattagataccctagtagtccacgccgtaaacgatgagtactaagtgttgggtgtcaaagctcagtgctgcagttaacgcaataagtactccgcctgagtagtacgttcgcaagaatgaaactcaaaggaattgacgggggcccgcacaagcggtggagcatgtggtttaattcgaagcaacgcgaagaaccttaccaggtcttgacatcgatctaaaggctccagagatggagagatagctatagagaagacaggtggtgcatggttgtcgtcagctcgtgtcgtgagatgttgggttaagtcccgcaacgagcgcaacccctgttgccagttgccagcattaagttggggactctggcgagactgccggtgacaagccggaggaaggcggggatgacgtcaaatcatcatgccccttatgacctgggctacacacgtgctacaatggacagagcagagggaagcgaagccgcgaggtggagcgaaacccataaaactgttctcagttcggactgcagtctgcaactcgactgcacgaagatggaatcgctagtaatcgcgaatcagcatgtcgcggtgaatacgttctcgggccttgtacacaccgcccgtcacaccatgagagtcggtaacacccgaagccggtggcctaaccgcaaggaaggagctgtctaaggtgggactgatgattggggtgaagtcgtaacaagggtaacc

SEQ ID NO: 25 - DNA, 1361 bp, HMI 26 Blautia luti 16S rDNA
  source 1..1361: mol_type = genomic DNA
cgggaatactttattgaaacttcggtggatttaatttatttctagtggcggacgggtgagtaacgcgtgggtaacctgccttatactgggggataacagccagaaatgactgctaataccgcataagcgcacagaaccgcatggttccgtgtgaaaaactccggtggtataagatggacccgcgttggattagctagttggcagggcagcggcctaccaaggcgacgatccatagccggcctgagagggtgaacggccacattgggactgagacacggcccagactcctacgggaggcagcagtggggaatattgcacaatgggggaaaccctgatgcagcgacgccgcgtgaaggaagaagtatctcggtatgtaaacttctatcagcagggaagataatgacggtacctgactaagaagccccggctaactacgtgccagcagccgcggtaatacgtagggggcaagcgttatccggatttactgggtgtaaagggagcgtagacggcgcagcaagtctgatgtgaaaggcaggggcttaacccctggactgcattggaaactgctgtgcttgagtgccggaggggtaagcggaattcctagtgtagcggtgaaatgcgtagatattaggaggaacaccagtggcgaaggcggcttactggacggtaactgacgttgaggctcgaaagcgtggggagcaaacaggattagataccctggtagtccacgccgtaaacgatgaatactaggtgtcagggagcacagctctttggtgccgccgcaaacgcattaagtattccacctggggagtacgttcgcaagaatgaaactcaaaggaattgacggggacccgcacaagcggtggagcatgtggtttaattcgaagcaacgcgaagaaccttaccaaatcttgacatccctctgaccgggacttaaccgtccctttccttcgggacaggggagacaggtggtgcatggttgtcgtcagctcgtgtcgtgagatgttgggttaagtcccgcaacgagcgcaacccctatccttagtagccagcacgtaatggtgggcactctgaggagactgccagggataacctggaggaaggcggggatgacgtcaaatcatcatgccccttatgatttgggctacacacgtgctacaatggcgtaaacaaagggaagcgaacccgcgagggtgggcaaatctcaaaaataacgtcccagttcggactgcagtctgcaactcgactgcacgaagctggaatcgctagtaatcgcggatcagaatgccgcggtgaatacgttcccgggtcttgtacacaccgcccgtcacaccatgggagtcagtaacgcccgaagtcag

SEQ ID NO: 26 - DNA, 1383 bp, HMI 27 Clostridium clostridioforme 16S rDNA
  source 1..1383: mol_type = genomic DNA
ttgcggtaggtcacaggcttcgggcatttccaactcccatggtgtgacgggcggtgtgtacaagacccgggaacgtattcaccgcgacatgctgattcgcgattactagcgattccagcttcatgtagtcgagttgcagactacaatccgaactgagacgttatttctgggatttgctcaacatcactgtctcgcttccctttgtttacgccattgtagcacgtgtgtagcccaaatcataaggggcatgatgatttgacgtcatccccgccttcctccgggttatccccggcagtctccctagagtgcccagctctacctgctggctactaaggataagggttgcgctcgttgcgggacttaacccaacatctcacgacacgagctgacgacaaccatgcaccacctgtctccaatgctccgaagagaatgccccgttacggacacgtcattgggatgtcaagacttggtaaggttcttcgcgttgcttcgaattaaaccacatgctccaccgcttgtgcgggtccccgtcaattcctttgagtttcattcttgcgaacgtactccccaggtggattgcttattgcgttagctgcggcaccgatgggtccatacccacctacacctagcaatcatcgtttaccgcgtggactaccagggtatctaatcctgtttgctccccacgctttcgagcctcaacgtcagttacagtccagtaagccgccttcgccactggtgttcctcctaatatctacgcatttcaccgctacactaggaattccgcttacctctcctgcactccagcctggcagttccaaatgcagtcccagggttgagccctgggttttcacatctggcttgtcatgccgtctacgctccctttacacccagtaaatccggataacgcttgccccctacgtattaccgcggctgctggcacgtagttagccggggcttcttagtcaggtaccgtcattttcttccctgctgatagagctttacataccgaaatacttcttcactcacgcggcgtcgctgcatcagggtttcccccattgtgcaatattccccactgctgcctcccgtaggagtttgggccgtgtctcagtcccaatgtggccgttcaccctctcaggccggctactgatcgtcgctttggtaggccgttaccctgccaactggctaatcagacgcgggaccatcctgtaccaccggagtttttcacactgcctcatgtgaagctgtgcgcttatgcggtattagcacctatttctaagtgttatcccccggtacagggcaggtttcccacgcgttactcacccgtccgccactaagttacgccgattccatccgaaaacttcctctgcataactccgtcgactg

SEQ ID NO: 27 - DNA, 1445 bp, HMI 28 Blautia producta 16S rDNA
  source 1..1445: mol_type = genomic DNA
ccggtggtcgcatcggcgctcctcctgtaggttgggtcactgacttcgggcgttactgactcccatggtgtgacgggcggtgtgtacaagacccgggaacgtattcaccgcgacattctgattcgcgattactagcgattccagcttcgtgcagtcgagttgcagactgcagtccgaactgggacgttatttttgggatttgctcaacatcgctgtctcgcttccctttgtttacgccattgtagcacgtgtgtagcccaaatcataaggggcatgatgatttgacgtcgtccccgccttcctccgggttatccccggcagtctccctagagtgcccagcttcacctgctggctactaaggataggggttgcgctcgttgcgggacttaacccaacatctcacgacacgagctgacgacaaccatgcaccacctgtctcctctgccccgaagggaaggccccgttacgggccggtcagagggatgtcaagacttggtaaggttcttcgcgttgcttcgaattaaaccacatgctccaccgcttgtgcgggtccccgtcaattcctttgagtttcattcttgcgaacgtactccccaggtggaatacttattgcgtttgctgcggcaccgaatgggctttgccacccgacacctagtattcatcgtttacggcgtggactaccagggtatctaatcctgtttgctccccacgctttcgagcctcaacgtcagttaccgtccagaaagccgccttcgccactggtgttcctcctaatatctacgcatttcaccgctacactaggaattccgcttacctctccggcactctagaaaaacagtttccaatgcagtcctggggttaagccccagcctttcacatcagacttgctcttccgtctacgctccctttacacccagtaaatccggataacgcttgccccctacgtattaccgcggctgatggcacgtagttagccggggcttcttagtcaggtaccgtcattttcttccctgctgatagaagtttacataccgagatacttcttccttcacgcggcgtcgctgcatcagggtttcccccattgtgcaatattccccactgctgcctcccgtaggagtctgggccgtgtctcagtcccaatgtggccgttcaccctctcaggccggctactgatcgtcgccttggtgggccgttacccctccaactagctaatcagacgcgggtccatctcataccaccggagtttttcacaccagaccatgcggtcctgtgcgcttatgcggtattagcagccatttctaactgttatccccctgtatgaggcaggttacccacgcgttactcagcccgtccgccgctcagtcaaataagtttcaatccgaagagatccacttaagtgcttcgctcgacttgcatgtgttaagcacgccgccagcgttcatcct

SEQ ID NO: 28 - DNA, 1412 bp, HMI 29 Blautia glucerasea 16S rDNA
  source 1..1412: mol_type = genomic DNA
gccttcggcagctccgtcctttcggttcggtcactgacttcgggcgttactgactcccatggtgtgacgggcggtgtgtacaagacccgggaacgtattcaccgcggcattctgatccgcgattactagcgattccagcttcgtgcagtcgagttgcagactgcagtccgaactgggacgttatttttgggatttgcttaagctcacactctcgcttccctttgtttacgccattgtagcacgtgtgtagcccaaatcataaggggcatgatgatttgacgtcatccccgccttcctccaggttatccctggcagtctcctcagagtgcccggccaaaccgctggctactaaggataggggttgcgctcgttgcgggacttaacccaacatctcacgacacgagctgacgacaaccatgcaccacctgtctccgatgctccgaagaaaaggcgacgttactcgccggtcatagggatgtcaagacttggtaaggttcttcgcgttgcttcgaattaaaccacatgctccaccgcttgtgcgggtccccgtcaattcctttgagtttcattcttgcgaacgtactccccaggtggaatacttactgcgtttgctgcggcaccgaatggctctgccacccgacacctagtattcatcgtttacggcgtggactaccagggtatctaatcctgtttgctccccacgctttcgagcctcaacgtcagttaccgtccagtaagccgccttcgccactggtgttcctcctaatatctacgcatttcaccgctacactaggaattccgcttacctctccggtactcaagatcaacagtttccaatgcagtccgggggttgagcccccgcctttcacatcagacttgctgctccgtctacgctccctttacacccagtaaatccggataacgcttgccccctacgtattaccgcggctgctggcacgtagttagccggggcttcttagtcaggtaccgtcattttcttccctgctgatagaagtttacataccgagatacttcttccttcacgcggcgtcgctgcatcagggtttcccccattgtgcaatattccccactgctgcctcccgtaggagtctgggccgtgtctcagtcccaatgtggccgtccaccctctcaggccggctatggatcgtcgctttggtaggccgttaccctgccaactggctaatccaacgcgggtccatctcacaccaccggagtttttcacactggatcatgcaatcccgtgcgcttatgcggtattagcagtcatttctgactgttatcccccagtgtgaggcaggttacccacgcgttactcacccgtccgccactaggattataacgacttcaaccgaagtctctgtcaaaataatccccgttcgacttgcatgtgt

SEQ ID NO: 29 - DNA, 1317 bp, HMI 30 Clostridium straminisolvens 16S rDNA
  source 1..1317: mol_type = genomic DNA
agcggcggacgggtgagtaacgcgtgagtaacctgcctttaggagggggacaacattccgaaagggatgctaataccgcataaaattattgtatcgcatggtataataatcaaagatttatcgcctaaagatggactcgcgtccgattagctagttggtggggtaaaagcctaccaaggcgacgatcggtagccgaactgagaggttgatcggccacattgggactgagacacggcccagactcctacgggaggcagcagtgggggatattgcgcaatgggggaaaccctgacgcagcaacgccgcgtgaaggaagaaggccttcgggttgtaaacttctttaagtgtggaagataatgacggtacacacagaataagccacggctaactacgtgccagcagccgcggtaatacgtaggtggcaagcgttgtccggatttactgggtgtaaagggcgtgtaggcgggtagacaagtcagatgtgaaataccggggctcaactccggggctgcatttgaaactgtatatcttgagtgtcggagaggaaagcggaattcctagtgtagcggtgaaatgcgtagatattaggaggaacaccagtggcgaaggcggctttctggacgataactgacgctgaggcgcgaaagcgtggggagcaaacaggattagataccctggtagtccacgccgtaaacgatggatactaggtgtaggaggtatcgaccccttctgtgccgcagttaacacaataagtatcccacctggggagtacggtcgcaagattgaaactcaaaggaattgacgggggcccgcacaagcagtggagtatgtggtttaattcgaagcaacgcgaagaaccttaccaggacttgacatcccacgcatagcctagagataggtgaagtcctacgggacgtggagacaggtggtgcatggttgtcgtcagctcgtgtcgtgagatgttgggttaagtcccgcaacgagcgcaacccttactgtcagttaccatcattaagttggggactctggcaggactgccggtgacaaatcggaggaaggtggggacgacgtcaaatcatcatgccccttatgtcctgggctacacacgtactacaatggctgttaacaaagtgaagcaaagcagtgatgtggagcaaaacacaaaaagcagtctcagttcagattgtaggctgaaactcgcctatatgaagtcggaattgctagtaatcgcagatcagcatgctgcggtgaatacgttcccgggccttgtacacaccgcccgtcacaccatgagagtcgataacacccgaagcctgt

SEQ ID NO: 30 - DNA, 1319 bp, HMI 31 Butyricoccus pullicaecorum 16S rDNA
  source 1..1319: mol_type = genomic DNA
agtggcggacgggtgagtaacgcgtgagcaatctgcctttaagagggggataacagtcggaaacggctgctaataccgcataaagcatcgaaaccgcatgattttgatgccaaaggagcaatccgcttttagatgagctcgcgtctgattagctggttggcggggtaacggcccaccaaggcgacgatcagtagccggactgagaggttgaacggccacattgggactgagacacggcccagactcctacgggaggcagcagtggggaatattgcgcaatgggggaaaccctgacgcagcaacgccgcgtgattgaagaaggccttcgggttgtaaagatctttaatcagggacgaaacaaatgacggtacctgaagaataagctccggctaactacgtgccagcagccgcggtaatacgtagggagcaagcgttatccggatttactgggtgtaaagggcgcgcaggcgggccggtaagttggaagtgaaatctatgggcttaacccataaactgcttttcaaactgctggtcttgagtgatggagaggcaggcggaattccgtgtgtagcggtgaaatgcgtagatatacggaggaacaccagtggcgaaggcggcctgctggacattaactgacgctgaggcgcgaaagcgtggggagcaaacaggattagataccctggtagtccacgccgtaaacgatggatactaggtgtgggaggtattgaccccttccgtgccgcagttaacacaataagtatcccacctggggagtacggccgcaaggttgaaactcaaaggaattgacgggggcccgcacaagcagtggagtatgtggtttaattcgaagcaacgcgaagaaccttaccaggtcttgacatcccgatgaccgcctcagagatgagccttttcttcggaacatcggtgacaggtggtgcatggttgtcgtcagctcgtgtcgtgagatgttgggttaagtcccgcaacgagcgcaacccttacggttagttgatacgcaagatcactctagccggactgccgttgacaaaacggaggaaggtggggacgacgtcaaatcatcatgccccttatgacctgggctacacacgtactacaatggcagtcatacagagggaagcaaaaccgcgaggtggagcaaatccctaaaagctgtcccagttcagattgcaggctgcaacccgcctgcatgaagtcggaattgctagtaatcgcggatcagcatgccgcggtgaatacgttcccgggccttgtacacaccgcccgtcacaccatgagagccgtcaatacccgaagtccgt

SEQ ID NO: 31 - DNA, 791 bp, HMI 32 Clostridium maritium 16S rDNA
  source 1..791: mol_type = genomic DNA
ctacactgcagtcgagcgatttcttcggtaagagcggcggacgggtgagtaacgcgtgggtaacctgccctatacacacggataacataccgaaaggtatgctaatacgagataacataagagattcgcatggatttcttatcaaagcttttgcggtataggatggacccgcgtctgattagctagttggtaaggtaacggcttaccaaggcgacgatcagtagccgacctgagagggtgatcggccacattggaactgagacacggtccaaactcctacgggaggcagcagtggggaatattgcacaatgggcgaaagcctgatgcagcaacgccgcgtgagcgatgaaggccttcgggtcgtaaagctctgtcctcaaggaagataatgacggtacttgaggaggaagccccggctaactacgtgccagcagccgcggtaatacgtagggggctagcgttatccggaattactgggcgtaaagggtgcgtaggtggtttcttaagtcagaggtgaaaggctacggctcaaccgtagtaagcctttgaaactgagaaacttgagtgcaggagaggagagtagaattcctagtgtagcggtgaaatgcgtagatattaggaggaataccagttgcgaaggcggctctctggactgtaactgacactgaggcacgaaagcgtggggagcaaacaggattagataccctggtagtccacgccgtaaacgatgagtactagctgtcggaggttacccccttcggtggcgcagctaacgcattaagtactccgcc

SEQ ID NO: 32 - DNA, 1377 bp, HMI 33 Eubacterium fissicatens 16S rDNA
  source 1..1377: mol_type = genomic DNA
agtggcggacgggtgagtaacgcgtgggtaacctgccttgtacagggggataacagttagaaatgactgctaataccgcataagcgcacagtatcgcatggtacagtgtgaaaaactccggtggtacaagatggacccgcgtctgattagctagttggtaaggtaacggcttaccaaggcaacgatcagtagccgacttgagagagtgatcggccacattgggactgagacacggcccaaactcctacgggaggcagcagtggggaatattgcacaatgggggaaaccctgatgcagcgacgccgcgtgagtgaagaagtatttcggtatgtaaaactctatcagcaaggaagataatgacggtacttgactaagaagccccggctaactacgtgccagcagccgcggtaatacgtagggggcaagcgttatccggatttactgggtgtaaagggagcgtagacggtatggtaagtcagatgtgaaagcccggggcttaaccccggaactgcatttgaaactatcaaactagagtgtcggagaggtaagtggaattcctagtgtagcggtgaaatgcgtagatattaggaggaacaccagtggcgaaggcggcttactggacgataactgacgttgaggctcgaaagcgtggggagcaaacaggattagataccctggtagtccacgccgtaaacgatgaatactaggtgtcagggaacaatagttctttggtgccgcagcaaacgcattaagtattccacctggggagtacgttcgcaagaatgaaactcaaaggaattgacggggacccgcacaagcggtggagcatgtggtttaattcgaagcaacgcgaagaaccttacctggtcttgacatcccaatgacgcctctttaatcggaggtttccttcgggacattggagacaggtggtgcatggttgtcgtcagctcgtgtcgtgagatgttgggttaagtcccgcaacgagcgcaacccttatctttagtagccagcagttcggctgggcactctagagagactgccagggataacctggaggaaggtggggatgacgtcaaatcatcatgccccttatgaccagggctacacacgtgctacaatggcgtaaacaaagggaagcaaaactgtgaggttgagcaaatcccaaaaataacgtctcagttcggattgtagtctgcaactcgactacatgaagctggaatcgctagtaatcgcagatcagaatgctgcggtgaatacgttcccgggtcttgtacacaccgcccgtcacaccatgggagtcggatatgcccgaagtcagtgacccaaccgtaaggagggagctgccgaaggtggagccgataactggggtgaagtcgt

SEQ ID NO: 33 - DNA, 1376 bp, HMI 34 Clostridium saccharolyticum 16S rDNA
  source 1..1376: mol_type = genomic DNA
agcggcggacgggtgagtaacgcgtgggtaacctgcctcatacagggggataacagttagaaatgactgctaataccgcataagcgcacagtgctgcatggcacagtgtgaaaaactccggtggtatgagatggacccgcgttggattaggcagttggcggggtaacggcccaccaaaccgacgatccatagccggcctgagagggtgaacggccacattgggactgagacacggcccaaactcctacgggaggcagcagtggggaatattgcacaatgggggaaaccctgatgcagcgacgccgcgtgagtgaagaagtaattcgttatgtaaagctctatcagcagggaagaaaatgacggtacctgactaagaagccccggctaactacgtgccagcagccgcggtaatacgtagggggcaagcgttatccggatttactgggtgtaaagggagcgtagacggccgtgcaagtctgatgtgaaaggctggggctcaaccccgggactgcattggaaactgtatggctggagtgccggagaggtaagcggaattcctagtgtagcggtgaaatgcgtagatattaggaggaacaccagtggcgaaggcggcttactggacggtaactgacgttgaggctcgaaagcgtggggagcaaacaggattagataccctggtagtccacgccgtaaacgatgattactaggtgttgggggacatggtccttcggtgccgccgcaaacgcagtaagtaatccacctggggagtacgttcgcaagaatgaaactcaaaggaattgacggggacccgcacaagcggtggagcatgtggtttaattcgaagcaacgcgaagaaccttaccaagtcttgacatcgagaggacagagtatgtaatgtactttcccttcggggcctcgaagacaggtggtgcatggttgtcgtcagctcgtgtcgtgagatgttgggttaagtcccgcaacgagcgcaacccctatcttcagtagccagcaattcggatgggcactctggagagactgccggggataacccggaggaaggcggggatgacgtcaaatcatcatgccccttatgacttgggctacacacgtgctacaatggcgtaaacaaagggaagcgagggagtgatccggagcaaatcccaaaaataacgtctcagttcggattgtagtctgcaactcgactacatgaagctggaatcgctagtaatcgcgaatcagcatgtcgcggtgaatacgttcccgggtcttgtacacaccgcccgtcacaccatgggagtcgataacgcccgaagtcagtgacccaaccgaaaggagggagctgccgaaggcgggattggtaactggggtgaagtcgt

SEQ ID NO: 34 - DNA, 1377 bp, HMI 35 Blautia luti 16S rDNA
  source 1..1377: mol_type = genomic DNA
agtggcggacgggtgagtaacgcgtgggtaacctgccttatactgggggataacagccagaaatggctgctaataccgcataagcgcacggggccgcatggtcctgtgtgaaaaactccggtggtataagatggacccgcgttggattagctagttggcagggcagcggcctaccaaggcgacgatccatagccggcctgagagggtgaacggccacattgggactgagacacggcccagactcctacgggaggcagcagtggggaatattgcacaatgggggaaaccctgatgcagcgacgccgcgtgaaggaagaagtatctcggtatgtaaacttctatcagcagggaagataatgacggtacctgactaagaagccccggctaactacgtgccagcagccgcggtaatacgtagggggcgagcgttatccggatttactgggtgtaaagggagcgtagacggcgtatcaagtctgatgtgaaaggcaggggcttaacccctggactgcattggaaactggtatgcttgagtgccggaggggtaagcggaattcctagtgtagcggtgaaatgcgtagatattaggaggaacaccagtggcgaaggcggcttactggacggtaactgacgttgaggctcgaaagcgtggggagcaaacaggattagataccctggtagtccacgccgtaaacgatgaatactaggtgtctgggagcacagctcttaggtgccgccgcaaacgcattaagtattccacctggggagtacgttcgcaagaatgaaactcaaaggaattgacggggacccgcacaagcggtggagcatgtggtttaattcgaagcaacgcgaagaaccttaccaaatcttgacatccctctgacagagtatgtaatgtacttttccttcgggacaggggagacaggtggtgcatggttgtcgtcagctcgtgtcgtgagatgttgggttaagtcccgcaacgagcgcaacccctatccttagtagccagcaagtaatgttgggcactctgaggagactgccagggataacctggaggaaggcggggatgacgtcaaatcatcatgccccttatgatttgggctacacacgtgctacaatggcgtaaacaaagggaagcgaacctgtgagggtgggcaaatctcaaaaataacgtcccagttcggactgcagtctgcaactcgactgcacgaagctggaatcgctagtaatcgcggatcagaatgccgcggtgaatacgttcccgggtcttgtacacaccgcccgtcacaccatgggagtcagtaacgcccgaagtcagtgacctaaccgtaaggaaggagctgccgaaggcgggacggatgactggggtgaagtcgt

SEQ ID NO: 35 - DNA, 1465 bp, HMI 36 Clostridium metylpentosum 16S rDNA
  source 1..1465: mol_type = genomic DNA
ggttaccttgttacgacttcaccccaatcatcaaccccaccttcgacgacgtcccccttgcggttagactatcggcttcgggtgttgccaactctcatggtgtgacgggcggtgtgtacaaggcccgggaacgtattcaccgcggcatgctgatccgcgattactagcaattccggcttcatgcaggcgggttgcagcctgcaatccgaactgagactatttttaggggtttgctccatgtcaccatcttgcttccctctgttaatagccattgtagtacgtgtgtagcccaggtcataaggggcatgatgatttgacgtcatccccaccttcctccgttttgtcaacggcagtccgtctagagtgctcttgcgtagcaactaaacgtaagggttgcgctcgttgcgggacttaacccaacatctcacgacacgagctgacgacaaccatgcaccacctgtctcggtgccccgaagggcttcacctatctctaggctatgcaccggatgtcaagacctggtaaggttcttcgcgttgcttcgaattaaaccacatactccactgcttgtgcgggcccccgtcaattcctttgagtttcaaccttgcggtcgtactccccaggtggattacttattgtgttaactccggcacggaaggggtcagtccccccacacctagtaatcatcgtttacagcgtggactaccagggtatctaatcctgtttgctacccacgctttcgagcctcagcgtcagttaaagcccagcaggccgccttcgccactggtgttcctcctaatatttacgcatttcaccgctacactaggaattccgcctgcctctacttcactcaagaactgcagttttgaacgcggctatgggttgagcccatagatttaacattcaacttgcaatcccgcctacgctccctttacacccagtaattccggacaacgctcgctacctacgtattaccgcggctgctggcacgtagttagccgtagcttcctccttggttaccgtcattatcttcaccaaggacagaggtttacaatccgaaaaccttcttccctcactcggcgtcgctgcatcagggtttcccccattgtgcaatattccccactgctgcctcccgtaggagtctgggccgtgtctcagtcccaatgtggccgttcaacctctcagtccggctaccaatcgtcgccttggtgggccgttacctcaccaactagctaattggacgcgagtccatctttcagcggattgctcctttgatatcagctccatgcgaaaccaatatgttatgcggtattagcgtccgtttccagacgttatccccctctgaaaggcaggttactcacgcgttactcacccgtccgccactaagttgaatcaaattccttccgaagaattcattcaaagcaacttcgtcgacttgcatgtgtaaggcgcgccgacagcgttcgt

SEQ ID NO: 36 - DNA, 1422 bp, HMI 37 Clostridium xylanolyticum 16S rDNA
  source 1..1422: mol_type = genomic DNA
agagtttgatcctggctcaggatgaacgctggcggcgtgcctaacacatgcaagtcgaacggaatttacatgaagcctagcgattgtaaatttagtggcggacgggtgagtaacgcgtgggtaacctgccttgtactgggggacaacagttggaaacgactgctaataccgcataagcgcacagcttcgcatgaagcagtgtgaaaaactccggtggtacaagatggacccgcgtctgattagctggttggtgaggtaacggcccaccaaggcgacgatcagtagccggcctgagagggtgaacggccacattgggactgagacacggcccaaactcctacgggaggcagcagtggggaatattgcacaatgggggaaaccctgatgcagcaacgccgcgtgagtgaagaagtatttcggtatgtaaagctctatcagcaggaaagaaaatgacggtacctgactaagaagccccggctaactacgtgccagcagccgcggtaatacgtagggggcaagcgttatccggatttactgggtgtaaagggagcgtagacggttttgcaagtctgaagtgaaagcccggggcttaaccccgggactgctttggaaactgtaggactagagtgcaggagaggtaagtggaattcctagtgtagcggtgaaatgcgtagatattaggaggaacaccagtggcgaaggcggcttactggactgtaactgacgttgaggctcgaaagcgtggggagcaaacaggattagataccctggtagtccacgccgtaaacgatgattactaggtgttggtgggtacgacccatcggtgccgcagcaaacgcaataagtaatccacctggggagtacgttcgcaagaatgaaactcaaaggaattgacggggacccgcacaagcggtggagcatgtggtttaattcgaagcaacgcgaagaaccttacctggtcttgacatccctatgaataacgggcaatgccgttagtacttcggtacataggagacaggtggtgcatggttgtcgtcagctcgtgtcgtgagatgttgggttaagtcccgcaacgagcgcaacccttatctttagtagccagcagtaagatgggcactctagagagactgccggggataacccggaggaaggtggggatgacgtcaaatcatcatgccccttatgaccagggctacacacgtgctacaatggcgtaaacaaagagaagcgaagtcgtgaggcagagcgaatctcaaaaataacgtctcagttcggattgtagtctgcaactcgactacatgaagctggaatcgctagtaatcgcagatcagaatgctgcggtgaatacgttcccgggtcttgtacacaccgcccgtcacaccatgggagtcggaaatgcccgaagtcggtgacctaaccgaa

SEQ ID NO: 37 - DNA, 1478 bp, HMI 38 Oscillibacter valericigenes 16S rDNA
  source 1..1478: mol_type = genomic DNA
ctcaggacgaacgctggcggcgtgcttaacacatgcaagtcgaacggagcacccttgactgaggtttcggccaaatgataggaatgcttagtggcggactggtgagtaacgcgtgaggaacctaccttccagagggggacaacagttggaaacgactgctaataccgcatgacgcatgaccggggcatcccgggcatgtcaaagattttatcgctggaagatggcctcgcgtctgattagctagatggtggggtaacggcccaccatggcgacgatcagtagccggactgagaggttgaccggccacattgggactgagatacggcccagactcctacgggaggcagcagtggggaatattgggcaatggacgcaagtctgacccagcaacgccgcgtgaaggaagaaggctttcgggttgtaaacttcttttgtcagggaagagtagaagacggtacctgacgaataagccacggctaactacgtgccagcagccgcggtaatacgtaggtggcaagcgttgtccggatttactgggtgtaaagggcgtgcagccgggccggcaagtcagatgtgaaatctggaggcttaacctccaaactgcatttgaaactgtaggtcttgagtaccggagaggttatcggaattccttgtgtagcggtgaaatgcgtagatataaggaagaacaccagtggcgaaggcggataactggacggcaactgacggtgaggcgcgaaagcgtggggagcaaacaggattagataccctggtagtccacgctgtaaacgatggatactaggtgtgcggggactgaccccctgcgtgccgcagttaacacaataagtatcccacctggggagtacgatcgcaaggttgaaactcaaaggaattgacgggggcccgcacaagcggtggattatgtggtttaattcgaagcaacgcgaagaaccttaccagggcttgacatcctactaacgaagtagagatacatcaggtgcccttcggggaaagtagagacaggtggtgcatggttgtcgtcagctcgtgtcgtgagatgttgggttaagtcccgcaacgagcgcaacccctattgttagttgctacgcaagagcactctagcgagactgccgttgacaaaacggaggaaggtggggacgacgtcaaatcatcatgccccttatgtcctgggctacacacgtaatacaatggcggtcaacagagggaggcaaagccgcgaggcagagcaaacccccaaaagccgtcccagttcggatcgcaggctgcaacccgcctgcgtgaagtcggaatcgctagtaatcgcggatcagcatgccgcggtgaatacgttcccgggccttgtacacaccgcccgtcacaccatgagagtcgggaacacccgaagtccgtagcctaaccgcaaggagggcgcggccgaaggtgggttcgataattggggtgaagtcgtaacaaggtaaccg

SEQ ID NO: 38 - DNA, 1620 bp, HMI 39 Ruminococcus obeum 16S rDNA
  source 1..1620: mol_type = genomic DNA
agtcgaacgggaaccttttattgaagcttcggcagatttagctggtttctagtggcggacgggtgagtaacgcgtgggtaacctgccctatacagggggataacaaccagaaatggttgctaataccgcataagcgcacaggaccgcatggtccggtgtgaaaaactccggtggtataggatggacccgcgttggattagccagttggcagggtaacggcctaccaaagcgacgatccatagccggcctgagagggtgaacggccacattgggactgagacacggcccagactcctacgggaggcagcagtggggaatattgcacaatgggggaaaccctgatgcagcgacgccgcgtgaaggaagaagtatctcggtatgtaaacttctatcagcagggaagatagtgacggtacctgactaagaagccccggctaactacgtgccagcagccgcggtaatacgtagggggcaagcgttatccggatttactgggtgtaaagggagcgtagacggattagcaagtctgatgtgaaaggcaggggctcaacccctggactgcattggaaactgccagtcttgagtgccggagaggtaagcggaattcctagtgtagcggtgaaatgcgtagatattaggaggaacaccagtggcgaaggcggcttactggacggcaactgacgttgaggctcgaaagcgtggggagcaaacaggattagataccctggtagtccacgccgtaaacgatgaatactaggtgttggggagcaaagctcttcggtgccgccgcaaacgcattaagtattccacctggggagtacgttcgcaagaatgaaactcaaaggaattgacggggacccgcacaagcggtggagcatgtggtttaattcgaagcaacgcgaagaaccttaccaagtcttgacatccctctgacggactcttaaccgagtctttccttcgggacagaggagacaggtggtgcatggttgtcgtcagctcgtgtcgtgagatgttgggttaagtcccgcaacgagcgcaacccctatccccagtagccagcatttcggatgggcactctgaggagactgccagggataacctggaggaaggcggggatgacgtcaaatcatcatgccccttatgatttgggctacacacgtgctacaatggcgtaaacaaagggaagcgagcctgcgagggtaagcaaatcccaaaaataacgtcccagttcggactgcagtctgcaactcgactgcacgaagctggaatcgctagtaatcgcggatcagaatgccgcggtgaatacgttcccgggtcttgtacacaccgcccgtcacaccatgggagtcagtaacgcccgaagtcagtgacctaaccgcaagggaggagctgccgaaggcgggaccgatgactggggtgaagtcgtaacaaggtaaccgtgactacacgaagctggaatcgctagtaatcgcggatcagaatgccgcggtgaatacgttcccgggtcttgtacacaccgcccgtcacaccatgggagtcagtaacgcccgaagtcagtgacctaaccgcaaggaaggagctgccgaaggcgggaccgatgactggggtgaagtcgtaaca

SEQ ID NO: 39 - DNA, 1403 bp, HMI 40 Megasphaera elsdenii 16S rDNA
  source 1..1403: mol_type = genomic DNA
acgcgtaagcaacctgccctccggatggggacaacagctggaaacggctgctaataccgaatacgtttccattgccgcatggcagtgggaagaaaggtggcctctgaatatgctaccgccgggggaggggcttgcgtctgattagctagttggaggggtaacggcccaccaaggcgacgatcagtagccggtctgagaggatgaacggccacattggaactgagacacggtccagactcctacgggaggcagcagtggggaatcttccgcaatgggcgaaagcctgacggagcaacgccgcgtgagcgaagacggccttcgggttgtaaagctctgttatacgggacgaacggctagtgtgccaataccacattagaatgacggtaccgtaagagaaagccacggctaactacgtgccagcagccgcggtaatacgtaggtggcaagcgttgtccggaattattgggcgtaaagggcgcgcaggcggtttcataagtctgtcttaaaagtgcggggcttaaccccgtgaggggacggaaactgtgagactggagtgtcggagaggaaagcggaattcctagtgtagcggtgaaatgcgtagatattaggaggaacaccagtggcgaaagcggctttctggacgacaactgacgctgaggcgcgaaagccaggggagcgaacgggattagataccccggtagtcctggccgtaaacgatggatactaggtgtagggggtatcgacccctcctgtgccggagttaacgcaataagtatcccgcctggggagtacggccgcaaggctgaaactcaaaggaattgacgggggcccgcacaagcggtggagtatgtggtttaattcgacgcaacgcgaagaaccttaccaagccttgacattgagtgctatcctcagagatgaggagttcttcttcggaagacgcgaaaacaggtggtgcacggctgtcgtcagctcgtgtcgtgagatgttgggttaagtcccgcaacgagcgcaacccctatcttctgttgccagcgcgtcatggcggggactcaggagagactgccgcagacaatgcggaggaaggcggggatgacgtcaagtcatcatgccccttatggcttgggctacacacgtactacaatggctcttaatagagggaagcgaaggagcgatccggagcaaaccccaaaaacagagtcccagttcggattgcaggctgcaacccgcctgcatgaagcaggaatcgctagtaatcgcaggtcagcatactgcggtgaatacgttcccgggccttgtacacaccgcccgtcacaccacgaaagtcattcacacccgaagccggtgaggtaaccgtaaggagccagccgtcgaaggtgggggcgatgattggggtgaagtcgtaa

SEQ ID NO: 40 - DNA, 1369 bp, HMI 41 Blautia luti 16S rDNA
  source 1..1369: mol_type = genomic DNA
ggtgagtaacgcgtgggtaacctgccttatacagggggataacagtcagaaatggctgctaataccgcataagcgcacagggccgcatggcccggtgtgaaaaactgaggtggtataagatggacccgcgttggattagccagttggcagggtaacggcctaccaaagcgacgatccatagccggcctgagagggtgaacggccacattgggactgagacacggcccagactcctacgggaggcagcagtggggaatattgcacaatgggggaaaccctgatgcagcgacgccgcgtgaaggaagaagtatctcggtatgtaaacttctatcagcagggaagaaaatgacggtacctgactaagaagccccggctaactacgtgccagcagccgcggtaatacgtagggggcaagcgttatccggatttactgggtgtaaagggagcgtagacggcataacaagtctgatgtgaaaggctggggcttaaccccgggactgcattggaaactgttaagcttgagtgccggaggggtaagcggaattcctagtgtagcggtgaaatgcgtagatattaggaggaacaccagtggcgaaggcggcttactggacggtaactgacgttgaggctcgaaagcgtggggagcaaacaggattagataccctggtagtccacgccgtaaacgatgaatactaggtgtcggggagcacagctcttcggtgccgccgcaaacgcattaagtattccacctggggagtacgttcgcaagaatgaaactcaaaggaattgacggggacccgcacaagcggtggagcatgtggtttaattcgaagcaacgcgaagaaccttaccaagtcttgacatctgcctgaccggtgagtaacgtcacctttccttcgggacaggcaagacaggtggtgcatggttgtcgtcagctcgtgtcgtgagatgttgggttaagtcccgcaacgagcgcaacccctatccccagtagccagcatgtaaaggtgggcactctgaggagactgccagggataacctggaggaaggtggggatgacgtcaaatcatcatgccccttatgatttgggctacacacgtgctacaatggcgtaaacagagggaagcgaaagggtgacctggagcaaatcccaaaaataacgtcccagttcggactgtagtctgcaacccgactacacgaagctggaatcgctagtaatcgcggatcagaatgccgcggtgaatacgttcccgggtcttgtacacaccgcccgtcacaccatgggagtcagtaacgcccgaagtcagtgacctaaccgaaagggaggagctgccgaaggcgggacggatgactggggtgaagtcgtaac

SEQ ID NO: 41 - DNA, 1359 bp, HMI 42 Bacteroides coprocola 16S rDNA
  source 1..1359: mol_type = genomic DNA
gtatccaaccttccgtttactcagggatagcctttcgaaagaaagattaatacctgatagtatggtaagattgcatgataataccattaaagattcatcggtaaacgatggggatgcgttccattaggtagtaggcggggtaacggcccacctagccgacgatggataggggttctgagaggaaggtcccccacattggaactgagacacggtccaaactcctacgggaggcagcagtgaggaatattggtcaatgggcgagagcctgaaccagccaagtagcgtgaaggatgaaggttctatggattgtaaacttcttttataagggaataaagtgctttacgtgtagagttttgtatgtaccttatgaataagcatcggctaactccgtgccagcagccgcggtaatacggaggatgcgagcgttatccggatttattgggtttaaagggagcgtagacgggatgttaagtcagctgtgaaagtttggggctcaaccttaaaattgcagttgaaactggcgttcttgagtgcggtagaggcaggcggaattcgtggtgtagcggtgaaatgcttagatatcacgaagaaccccgattgcgaaggcagcttgctggagcgtaactgacgttgatgctcgaaagtgtgggtatcaaacaggattagataccctggtagtccacacggtaaacgatggatactcgctgttggcgatatacggtcagcggccaagcgaaagcattaagtatcccacctggggagtacgccggcaacggtgaaactcaaaggaattgacgggggcccgcacaagcggaggaacatgtggtttaattcgatgatacgcgaggaaccttacccgggcttaaattatgcatgaatgatctggagacagatcagccgcaaggcatgtatgaaggtgctgcatggttgtcgtcagctcgtgccgtgaggtgtcggcttaagtgccataacgagcgcaaccctttctgccagttactaacaggcaatgctgaggactctggcggtactgccatcgtaagatgtgaggaaggtggggatgacgtcaaatcagcacggcccttacgtccggggctacacacgtgttacaatggggggtacagaaggcagcttaccggcgacggttggccaatccctaaagcccctctcagttcggactggagtctgcaacccgactccacgaagctggattcgctagtaatcgcgcatcagccacggcgcggtgaatacgttcccgggccttgtacacaccgcccgtcaagccatgaaagccgggagtacctgaagtgcgtaaccgcgaggagcgccctagggtaacactggtaattggggctaagtcgt

SEQ ID NO: 42 - DNA, 1406 bp, HMI 43 Bacteroides plebius 16S rDNA
  source 1..1406: mol_type = genomic DNA
ggggcagcatgaacttagcttgctaagttcgatggcgaccggcgcaccgttgagtaacgcgtatccaaccttccgtacactcaggaatagcctttcgaaagaaagattaatacctgatggtatgatgggattgcatgaaatcatcattaaagattcatcggtgtacgatggggatgcgttccattagatagtaggcggggtaacggcccacctagtcgacgatggataggggttctgagaggaaggtcccccacattggaactgagacacggtccaaactcctacgggaggcagcagtgaggaatattggtcaatgggcgcgagcctgaaccagccaagtagcgtgaaggatgaaggtcctacggattgtaaacttcttttataagggaataaagtcacccacgtgtgggtgtttgtatgtaccttatgaataagcatcggctaactccgtgccagcagccgcggtaatacggaggatgcgagcgttatccggatttattgggtttaaagggagcgtagacgggtcgttaagtcagctgtgaaagttcggggctcaaccttgaaattgcagttgatactggcgtccttgagtacggttgaggcaggcggaattcgtggtgtagcggtgaaatgcttagatatcacgaagaaccccgattgcgaaggcagcctgctaaaccgccactgacgttgaggctcgaaagtgtgggtatcaaacaggattagataccctggtagtccacacggtaaacgatggatactcgctgttggcgatagactgtcagcggcttagcgaaagcgttaagtatcccacctggggagtacgccggcaacggtgaaactcaaaggaattgacgggggcccgcacaagcggaggaacatgtggtttaattcgatgatacgcgaggaaccttacccgggcttgaattgcagacgaattgcttggaaacaggcaagccgcaaggcgtctgtgaaggtgctgcatggttgtcgtcagctcgtgccgtgaggtgtcggcttaagtgccataacgagcgcaaccctcgtgtccagttgctagcaggtagtgctgaggactctggacagactgccatcgtaagatgtgaggaaggtggggatgacgtcaaatcagcacggcccttacgtccggggctacacacgtgttacaatggggggtacagcaggcagctaccgggcgaccggatgccaatcccgaaagcctctctcagttcggactggagtctgcaacccgactccacgaagctggattcgctagtaatcgcgcatcagccacggcgcggtgaatacgttcccgggccttgtacacaccgcccgtcaagccatgaaagccgggggtacctgaagtgcgtaaccgcaaggagcgccctagggtaaaactggtaatt

SEQ ID NO: 43 - DNA, 1420 bp, HMI 44 Roseburia inulinivorans 16S rDNA
  source 1..1420: mol_type = genomic DNA
gcacttttgccgattttcttcggaactgaagtaatagtgactgagtggcggacgggtgagtaacgcgtggataacctgcctcacacagggggataacagttagaaatgactgctaataccgcataagcgcacagtaccgcatggtacagtgtgaaaaactccggtggtgtgagatggatccgcgtctgattagccagttggcggggtaacggcccaccaaagcgacgatcagtagccggcctgagagggcgaccggccacattgggactgagacacggcccagactcctacgggaggcagcagtggggaatattgcacaatgggggaaaccctgatgcagcgacgccgcgtgagcgaagaagtatttcggtatgtaaagctctatcagcagggaagaaaatgacggtacctgactaagaagctccggctaaatacgtgccagcagccgcggtaatacgtatggagcaagcgttatccggatttactgggtgtaaagggagcgcaggcggtatgacaagtctgatgtgaaaggctggggctcaaccccaggactgcattggaaactgtcagactagagtgtcggagaggtaagtggaattcctagtgtagcggtgaaatgcgtagatattaggaggaacaccagtggcgaaggcggcttactggacgacaactgacgctgaggctcgaaagcgtggggagcaaacaggattagataccctggtagtccacgccgtaaacgatgaatactaggtgtcgggaggcagagcctttcggtgccgcagcaaacgcagtaagtattccacctggggagtacgttcgcaagaatgaaactcaaaggaattgacggggacccgcacaagcggtggagcatgtggtttaattcgaagcaacgcgaagaaccttaccaggccttgacatccccctgacgggacagtaatgtgtccgttccttcgggacagaggagacaggtggtgcatggttgtcgtcagctcgtgtcgtgagatgttgggttaagtcccgcaacgagcgcaacccttatcctcagtagccagcggataaagccgggcactctgtggagactgccagggacaacctggaggaaggtggggatgacgtcaaatcatcatgccccttatggcctgggctacacacgtgctacaatggcgtaaacaaagggaagcgaagctgtgaagtgaagcaaatcccaaaaataacgtctcagttcggattgtagtctgcaactcgactacatgaagctggaatcgctagtaatcgcgaatcagaatgtcgcggtgaatacgttcccgggtcttgtacacaccgcccgtcacaccatgggagtcgggaatgcccgaagccggtgacccaaccttaaggagggagccgtcgaaggcaggcctgataactggggtgaagtcgt

SEQ ID NO: 44 - DNA, 1392 bp, HMI 45 Ruminococcus albus 16S rDNA
  source 1..1392: mol_type = genomic DNA
ctgatctagtggcggacgggtgagtaacacgtgagcaatctgcctttcagagggggataccgattggaaacgatcgttaataccgcataacataattgaaccgcatgatttgattatcaaagatttatcgctgaaagatgagctcgcgtctgattagctagttggtaaggtaacggcttaccaaggcgacgatcagtagccggactgagaggttgatcggccacattgggactgagacacggcccagactcctacgggaggcagcagtggggaatattgcacaatggaggaaactctgatgcagcgatgccgcgtgagggaagaaggttttaggattgtaaacctctgtcttcagggacgaaaaaagacggtacctgaggaggaagctccggctaactacgtgccagcagccgcggtaatacgtagggagcgagcgttgtccggaattactgggtgtaaagggagcgtaggcgggatcgcaagtcagatgtgaaaactatgggcttaacccataaactgcatttgaaactgtggttcttgagtgaagtagaggtaagcggaattcctagtgtagcggtgaaatgcgtagatattaggaggaacatcagtggcgaaggcggcttactgggctttaactgacgctgaggctcgaaagcgtggggagcaaacaggattagataccctggtagtccacgccgtaaacgatgattactaggtgtggggggactgaccccttccgtgccgcagcaaacgcaataagtaatccacctggggagtacgaccgcaaggttgaaactcaaaggaattgacgggggcccgcacaagcagtggagtatgtggattaattcgaagcaacgcgaagaaccttaccaggtcttgacatcgtatgcatagctcagagatgagtgaaatctcttcggagacatatagacaggtggtgcatggttgtcgtcagctcgtgtcgtgagatgttgggttaagtcccgcaacgagcgcaacccttactgttagttgctacgcaagagcactctagcaggactgccgttgacaaaacggaggaaggtggggatgacgtcaaatcatcatgccccttatgacctgggcctcacacgtactacaatggctgttaacagagggatgcaaagccgcgaggtagagcgaacccctaaaagcagtcttagttcggattgtaggctgcaacccgcctacatgaagtcggaattgctagtaatcgcagatcagcatgctgcggtgaatacgttcccgggccttgtacacaccgcccgtcacgccatgggagtcggtaacacccgaagcctgtagtctaaccgcaaggaggacgcagtcgaaggtgggattgatgactggggtgaagtcgtaacagggtaaccg

SEQ ID NO: 45 - DNA, 1414 bp, HMI 46 Blautia producta 16S rDNA
  source 1..1414: mol_type = genomic DNA
tggacagattcttcggatgaagtccttagtgactgagtggcggacgggtgagtaacgcgtgggtaacctgcctcatacagggggataacagttagaaatggctgctaataccgcataagcgcacggtactgcatggtacagtgtgaaaaactccggtggtatgagatggacccgcgttggattagctagttggcagggtaacggcctaccaaggcgacgatccatagccggcctgagagggtggacggccacattgggactgagacacggcccagactcctacgggaggcagcagtggggaatattgcacaatgggggaaaccctgatgcagcgacgccgcgtgagcgaagaagtatttcggtatgtaaagctctatcagcagggaagaaaatgacggtacctgactaagaagccccggctaactacgtgccagcagccgcggtaatacgtagggggcaagcgttatccggatttactgggtgtaaagggagcgtagacggaatggcaagtctgatgtgaaaggccggggctcaaccccgggactgcattggaaactgtcaatctagagtaccggaggggtaagtggaattcctagtgtagcggtgaaatgcgtagatattaggaggaacaccagtggcgaaggcggcttactggacggtaactgacgttgaggctcgaaagcgtggggagcaaacaggattagataccctggtagtccacgccgtaaacgatgaatactaggtgttggggagcaaagctcttcggtgccgcagcaaacgcaataagtattccacctggggagtacgttcgcaagaatgaaactcaaaggaattgacggggacccgcacaagcggtggagcatgtggtttaattcgaagcaacgcgaagaaccttaccaaatcttgacatcgatctgaccggactgtaatgagtcctttcccttcggggacagagaagacaggtggtgcatggttgtcgtcagctcgtgtcgtgagatgttgggttaagtcccgcaacgagcgcaacccttatcctcagtagccagcaagtgaagttgggcactctgtggagactgccagggataacctggaggaaggtggggatgacgtcaaatcatcatgccccttatgatttgggctacacacgtgctacaatggcgtaaacaaagggaagcgatcacgcgagtgtgagcaaatctcaaaaataacgtctcagttcggattgtagtctgcaactcgactacatgaagctggaatcgctagtaatcgcaggtcagcatactgcggtgaatacgttcccgggtcttgtacacaccgcccgtcacaccatgggagtcagtaacacccgaagccggtgacctaaccgaaaggaaggagccgtcgaaggtgggaccgataactggggtgaagtcgt

SEQ ID NO: 46 - DNA, 1389 bp, HMI 47 Clostridium nexile 16S rDNA
  source 1..1389: mol_type = genomic DNA
gtttgtgacttagtggcggacgggtgagtaacgcgtgggtaacctgccttatacagggggataacagttagaaatgactgctaataccgcataagcgcacagtctcgcatgggacagtgtgaaaaactaaggtggtataagatggacccgcgtctgattagctagttggtggggtaaaggcctaccaaggcgacgatcagtagccgacctgagagggtgatcggccacattgggactgagacacggcccaaactcctacgggaggcagcagtggggaatattgcacaatgggggaaaccctgatgcagcaacgccgcgtgaaggaagaagtatctcggtatgtaaacttctatcagcagggaagaaaatgacggtacctgactaagaagctccggctaaatacgtgccagcagccgcggtaatacgtatggagcaagcgttatccggatttactgggtgtaaagggagcgtaggcggttatgcaagtcagatgtgaaagcccggggcttaaccccgggactgcatttgaaactgtgtaactagagtgtcggagaggtaagtggaattcctagtgtagcggtgaaatgcgtagatattaggaggaacaccagtggcgaaggcggcttactggacgataactgacgctgaggctcgaaagcgtggggagcaaacaggattagataccctggtagtccacgccgtaaacgatgaatactaggtgttggggagcaaagctcttcggtgccgcagcaaacgcaataagtattccacctggggagtacgttcgcaagaatgaaactcaaaggaattgacggggacccgcacaagcggtggagcatgtggtttaattcgaagcaacgcgaagaaccttaccaagtcttgacatctggatgaccggaccgtaatgggtcctttccttcgggacatccaagacaggtggtgcatggttgtcgtcagctcgtgtcgtgagatgttgggttaagtcccgcaacgagcgcaacccttatccttagtagccagcagtaagatgggcactctagggagactgccggagacaatccggaggaaggtggggatgacgtcaaatcatcatgccccttatgacttgggctacacacgtgctacaatggcgtaaacaaagggaagcgagaccgcgaggttaagcaaatctcaaaaataacgtctcagttcggattgtagtctgcaactcgactacatgaagctggaatcgctagtaatcgcgaatcagcatgtcgcggtgaatacgttcccgggtcttgtacacaccgcccgtcacaccatgggagtcgataacgcccgaagccggtgactcaaccgaaaggagagagccgtcgaaggcgggatggataactggggtgaagtcgtaac

SEQ ID NO: 47 - DNA, 1404 bp, HMI 48 Butyricicoccus pullicaecorum 16S rDNA
  source 1..1404: mol_type = genomic DNA
atctcttcggagatggaattcttaacctagtggcggacgggtgagtaacgcgtgagcaatctgcctttaggagggggataacagtcggaaacggctgctaataccgcataatacgtttgggaggcatctcttgaacgtcaaagattttatcgcctttagatgagctcgcgtctgattagctggttggcggggtaacggcccaccaaggcgacgatcagtagccggactgagaggttgaacggccacattgggactgagacacggcccagactcctacgggaggcagcagtggggaatattgcgcaatgggggaaaccctgacgcagcaacgccgcgtgattgaagaaggccttcgggttgtaaagatctttaatcagggacgaaaaatgacggtacctgaagaataagctccggctaactacgtgccagcagccgcggtaatacgtagggagcaagcgttatccggatttactgggtgtaaagggcgcgcaggcgggccggcaagttgggagtgaaatcccggggcttaaccccggaactgctttcaaaactgctggtcttgagtgatggagaggcaggcggaattccgtgtgtagcggtgaaatgcgtagatatacggaggaacaccagtggcgaaggcggcctgctggacattaactgacgctgaggcgcgaaagcgtggggagcaaacaggattagataccctggtagtccacgccgtaaacgatggatactaggtgtgggaggtattgaccccttccgtgccgcagttaacacaataagtatcccacctggggagtacggccgcaaggttgaaactcaaaggaattgacgggggcccgcacaagcagtggagtatgtggtttaattcgaagcaacgcgaagaaccttaccaggtcttgacatcccgatgaccggcgtagagatacgccctctcttcggagcatcggtgacaggtggtgcatggttgtcgtcagctcgtgtcgtgagatgttgggttaagtcccgcaacgagcgcaacccttacggttagttgatacgcaagatcactctagccggactgccgttgacaaaacggaggaaggtggggacgacgtcaaatcatcatgccccttatgacctgggctacacacgtactacaatggcagtcatacagagggaagcaataccgcgaggtggagcaaatccctaaaagctgtcccagttcagattgcaggctgcaacccgcctgcatgaagtcggaattgctagtaatcgcggatcagcatgccgcggtgaatacgttcccgggccttgtacacaccgcccgtcacaccatgagagccgtcaatacccgaagtccgtagcctaaccgcaaggggggcgcggccgaaggtaggggtggtaattagggtgaagtcgtac

SEQ ID NO: 48 - DNA, 1407 bp, HMI 49 Ruminococcus flavefaciens 16S rDNA
  source 1..1407: mol_type = genomic DNA
agtcgacggacgaggaggagcttgcttctccgagttagtggcggacgggtgagtaacacgtgagcaacctacccttgagagggggatagcttctggaaacggatggtaataccccataacatatattttaggcatctaagatatatcaaagaaattcgctcaaggatgggctcgcgtctgattagatagttggtgaggtaacggcccaccaagtcgacgatcagtagccggactgagaggttgaacggccacattgggactgagacacggcccagactcctacgggaggcagcagtggggaatattgcacaatggggggaaccctgatgcagcgatgccgcgtggaggaagaaggttttcggattgtaaactccttttaacagggacgataatgacggtacctgaagaaaaagctccggctaactacgtgccagcagccgcggtaatacgtagggagcgagcgttgtccggaattactgggtgtaaagggagcgtaggcgggacggtaagtcaggtgtgaaatatacgtgctcaacatgtagactgcacttgaaactgctgttcttgagtgaagtagaggtaagcggaattcctagtgtagcggtgaaatgcgtagatattaggaggaacatcggtggcgaaggcggcttactgggcttttactgacgctgaggctcgaaagcgtggggagcaaacaggattagataccctggtagtccacgctgtaaacgatgattactaggtgtggggggactgaccccttccgtgccgcagttaacacaataagtaatccacctggggagtacgaccgcaaggttgaaactcaaaggaattgacgggggcccgcacaagcagtggagtatgtggtttaattcgaagcaacgcgaagaaccttaccaggtcttgacatcgtatgcatagtctagagatagatgaaatcccttcggggacatatagacaggtggtgcatggttgtcgtcagctcgtgtcgtgagatgttgggttaagtcccgcaacgagcgcaacccttacctttagttgctacgcaagagcactctagagggactgccgttgacaaaacggaggaaggtggggatgacgtcaaatcatcatgccccttatgacctgggctacacacgtactacaatggcaattaacagagggaagcaaaacagcgatgtggagcaaatcccgaaaaattgtcccagttcagattgcaggctgcaactcgcctgcatgaagtcggaattgctagtaatcgcagatcagaatgctgcggtgaatacgttcccgggccttgtacacaccgcccgtcacaccatgggagtcggtaacacccgaagcctgtagtctaaccttataggaggacgcagtcgaaggtgggattgatgactggggtgaagtcgt

SEQ ID NO: 49 - DNA, 1349 bp, HMI 50 Clostridium orbiscindens 16S rDNA
  source 1..1349: mol_type = genomic DNA
aaagggaatgcttagtggcggacgggtgagtaacgcgtgagtaacctgccttggagtggggaataacagccggaaacggctgctaataccgcatgatgtatctggatcgcatggttctggataccaaagatttatcgctctgagatggactcgcgtctgattagctagttggtgaggtaacggctcaccaaggcgacgatcagtagccggactgagaggttggccggccacattgggactgagacacggcccagactcctacgggaggcagcagtggggaatattgggcaatgggcgaaagcctgacccagcaacgccgcgtgaaggaagaaggccctcgggttgtaaacttcttttgtcagggacgaagcaagtgacggtacctgacgaataagccacggctaactacgtgccagcagccgcggtaatacgtaggtggcaagcgttatccggatttactgggtgtaaagggcgtgtaggcgggagtgcaagtcagatgtgaaaactatgggctcaacccatagcctgcatttgaaactgtacttcttgagtgatggagaggcaggcggaattccctgtgtagcggtgaaatgcgtagatatagggaggaacaccagtggcgaaggcggcctgctggacattaactgacgctgaggcgcgaaagcgtggggagcaaacaggattagataccctggtagtccacgccgtaaacgatggatactaggtgtggggggtctgaccccctccgtgccgcagttaacacaataagtatcccacctggggagtacgatcgcaaggttgaaactcaaaggaattgacgggggcccgcacaagcggtggagtatgtggtttaattcgaagcaacgcgaagaaccttaccaggacttgacatcctactaacgaagcagagatgcataaggtgcccttcggggaaagtagagacaggtggtgcatggttgtcgtcagctcgtgtcgtgagatgttgggttaagtcccgcaacgagcgcaacccttattgttagttgctacgcaagagcactctagcgagactgccgttgacaaaacggaggaaggtggggacgacgtcaaatcatcatgccccttatgtcctgggccacacacgtactacaatggcggtcaacagagggaagcaaagccgcgaggtggagcaaatccctaaaagccgtcccagttcggattgcaggctgaaactcgcctgtatgaagtcggaatcgctagtaatcgcggatcagcatgccgcggtgaatacgttcccgggccttgtacacaccgcccgtcacaccatgagagtcgggaacacccgaagtccgtagcctaacagcaatggg

SEQ ID NO: 50 - DNA, 1420 bp, HMI 51 Ruminococcus bromii 16S rDNA
  source 1..1420: mol_type = genomic DNA
acgaagctttgaggagcttgctttttaagcttagtggcggacgggtgagtaacgcgtgagcaacctgcctctcagaggggaataacgttttgaaaagaacgctaataccgcataacatatcggaaccgcatgattctgatatcaaaggagcaatccgctgagagatgggctcgcgtccgattagttagttggtgaggtaacggctcaccaagactacgatcggtagccggactgagaggttgatcggccacattgggactgagacacggcccagactcctacgggaggcagcagtgggggatattgcgcaatgggggaaaccctgacgcagcaacgccgcgtgaaggaagaaggtcttcggattgtaaacttcttttgtcagggacgaagaaagtgacggtacctgacgaataagctccggctaactacgtgccagcagccgcggtaatacgtagggagcgagcgttgtccggatttactgggtgtaaagggtgcgtaggcggccgagcaagtcagttgtgaaaactatgggcttaacccataacgtgcaattgaaactgtccggcttgagtgaagtagaggtaggcggaattcccggtgtagcggtgaaatgcgtagagatcgggaggaacaccagtggcgaaggcggcctactgggctttaactgacgctgaggcacgaaagcatgggtagcaaacaggattagataccctggtagtccatgccgtaaacgatgattactaggtgtggggggactgaccccttccgtgccgcagttaacacaataagtaatccacctggggagtacggccgcaaggttgaaactcaaaggaattgacgggggcccgcacaagcagtggagtatgtggtttaattcgaagcaacgcgaagaaccttaccaggtcttgacatcctgagaatccttaagagattagggagtgccttcgggaactcagagacaggtggtgcatggttgtcgtcagctcgtgtcgtgagatgttgggttaagtcccgcaacgagcgcaacccttgctattagttgctacgcaagagcactctaataggactgccgttgacaaaacggaggaaggtggggacgacgtcaaatcatcatgccccttatgacctgggctacacacgtactacaatggccattaacagagggaagcaaaaccgcgaggcagagcaaacccctaaaaatggtcccagttcggattgtaggctgcaacccgcctacatgaagttggaattgctagtaatcgcggatcagcatgccgcggtgaatacgttcccgggccttgtacacaccgcccgtcacaccatgggagccggtaatacccgaagtcagtagtctaacagcaatgaggacgctgccgaaggtaggattggcgactggggtgaagtcgtaacaaggtaaccg

SEQ ID NO: 51 - DNA, 1490 bp, HMI 52 Ruminococcus albus 926R 16S rDNA
  source 1..1490: mol_type = genomic DNA
agagtttgatcctggctcaggacgaacgctggcggcacgcttaacacatgcaagtcgaacgagagaagagaagcttgcttttctgatctagtggcggacgggtgagtaacacgtgagcaatctgcctttcagagggggataccgattggaaacgatcgttaataccgcataacataattgaaccgcatgatttgattatcaaagatttatcgctgaaagatgagctcgcgtctgattagctagttggtaaggtaacggcttaccaaggcgacgatcagtagccggactgagaggttgatcggccacattgggactgagacacggcccagactcctacgggaggcagcagtggggaatattgcacaatggaggaaactctgatgcagcgatgccgcgtgagggaagaaggttttaggattgtaaacctctgtcttcagggacgaaaaaaaagacggtacctgaggaggaagctccggctaactacgtgccagcagccgcggtaatacgtagggagcgagcgttgtccggaattactgggtgtaaagggagcgtaggcgggatcgcaagtcagatgtgaaaactatgggcttaacccataaactgcatttgaaactgtggttcttgagtgaagtagaggtaagcggaattcctagtgtagcggtgaaatgcgtagatattaggaggaacatcagtggcgaaggcggcttactgggctttaactgacgctgaggctcgaaagcgtggggagcaaacaggattagataccctggtagtccacgccgtaaacgatgattactaggtgtggggggactgaccccttccgtgccgcagcaaacgcaataagtaatccacctggggagtacgaccgcaaggttgaaactcaaaggaattgacgggggcccgcacaagcagtggagtatgtggattaattcgaagcaacgcgaagaaccttaccaggtcttgacatcgtatgcatagctcagagatgagtgaaatctcttcggagacatatagacaggtggtgcatggttgtcgtcagctcgtgtcgtgagatgttgggttaagtcccgcaacgagcgcaacccttactgttagttgctacgcaagagcactctagcaggactgccgttgacaaaacggaggaaggtggggatgacgtcaaatcatcatgccccttatgacctgggcctcacacgtactacaatggctgtcaacagagggatgcaaagccgcgaggtggagcgaacccctaaaagcagtcttagttcggattgtaggctgcaacccgcctacatgaagtcggaattgctagtaatcgcagatcagcatgctgcggtgaatacgttcccgggccttgtacacaccgcccgtcacgccatgggagtcggtaacacccgaagcctgtagtctaaccgcaaggaggacgcagtcgaaggtgggattgatgactggggtgaagtcgtaacaaggtagccgtatcggaaggtgcg